European Patent Specification EP 3 611 192 B1, published March 5, 2025. Title: T CELL RECRUITING POLYPEPTIDES BASED ON TCR ALPHA/BETA REACTIVITY. Applicant: Ablynx N.V. The sequence listing filed with the application follows.

SEQUENCE LISTING (487 sequences)

SEQ ID NO: 1 - protein, 117 aa, Artificial Sequence
  Nanobody sequence
EVQLVESGGGLVQPGGSLRLSCAASGSVHKINFLGWYRQAPGKERELVATITIGDTTDYADSAKGRFTISRDEAKNMVYLQMNSLKPEDTAVHFCRAGSRLYPYNYWGQGTQVTVSS

SEQ ID NO: 2 - protein, 117 aa, Artificial Sequence
  Nanobody sequence
EVQLVESGGGLVQPGGSLRLSCAASGSVHKINFLGWYRQAPGKERGLVATITIGDTTDYADYAKGRFTISRDEARNMVYLQMNSLKPEDTAVYFCRAGSRLYPYNYWGQGTQVTVSS

SEQ ID NO: 3 - protein, 117 aa, Artificial Sequence
  Nanobody sequence
EVQLVESGGGLVQPGRSLRLPCAASGSVHKINFLGWYRQAPGKEREMVATITIGDATDYADSAKGRFTISRDEAKNMVYLQMNSLKPEDTAVYFCRAGSRLYPYNYWGQGTQVTVSS

SEQ ID NO: 4 - protein, 117 aa, Artificial Sequence
  Nanobody sequence
EVQLVESGGGLVQPGGSLRLSCAASGSVHKINFLGWYRQAPGKERELVATITIGDTTDYADYAKGRFTISRDEARNMVYLQMNSLKPEDTAVYFCRAGSRLYPYNYWGQGTLVTVSS

SEQ ID NO: 5 - protein, 117 aa, Artificial Sequence
  Nanobody sequence
EVQLVESGGGLVQPGGSLRLSCAASGSVHKINFLGWYRQAPGKEREMVATITIGDATDYADSAKGRFTISRDEAKNMVYLQMNSLKPEDTAVYFCRAGSRLYPYNYWGQGTLVTVSS

SEQ ID NO: 6 - protein, 117 aa, Artificial Sequence
  Nanobody sequence
EVQLVESGGGLVQPGGSLRLSCAASGSVHKINFLGWYRQAPGKERELVATITIGDTTDYADSAKGRFTISRDEAKNMVYLQMNSLKPEDTAVYFCRAGSRLYPYNYWGQGTQVTVSS

SEQ ID NO: 7 - protein, 117 aa, Artificial Sequence
  Nanobody sequence
EVQLVESGGGLVQPGGSLRLSCAVSGSVHLLNFLGWYRQAPGKEREMVAHITIADATDYSHFAKGRFTISRDEAKNMVYLQMNSLRPEDTAVYFCRAGSRIYPYDYWGQGTLVTVSS

SEQ ID NO: 8 - protein, 117 aa, Artificial Sequence
  Nanobody sequence
EVQLVESGGGLVQPGGSLKLSCAASGAVHKINFLGWYRQTPEKEREMVATITIGDDVDYADSAKGRFTISRDEAKNMVYLQMTSLKPEDTAVYVCRAGSRLYPYNYWGQGTLVTVSS

SEQ ID NO: 9 - protein, 117 aa, Artificial Sequence
  Nanobody sequence
EVQLVESGGGLVQPGGSLRLSCRASGDVHKINILGWYRQAPAKEREMVAHITIGDATDYAESAKGRFTISRDEAKNMVYLQMNSLKPEDTAVYFCRAYSRIYPYNYWGQGTQVTVSS

SEQ ID NO: 10 - protein, 117 aa, Artificial Sequence
  Nanobody sequence
EVQLVESGGGLVRPGGSLRLSCAASGDVHKINILGWYRQAPAKEREMVAHITIGDATDYADSAKGRFTISRDEAKNMVYLQMNSLKPEDTAVYFCRAYSRIYPYNYWGQGTLVTVSS

SEQ ID NO: 11 - protein, 117 aa, Artificial Sequence
  Nanobody sequence
EVQLVESGGGLVQPGGSLRLSCAASGDVHKINILGWYRQAPAKEREMVAHITIGDATDYADSAKGRFTISRDEAKNMVYLQMNSLKPEDTAVYFCRAYSRIYPYNYWGQGTLVTVSS

SEQ ID NO: 12 - protein, 117 aa, Artificial Sequence
  Nanobody sequence
EVQLVESGGGLVQPGGSLRLSCVASGDVHKINFLGWYRQAPGKEREKVAHITIGDQADYADSAKGRFTISRDEAKNMVYLQMNSLKPEDTAVYFCRAGSRIYPYDYWGQGTQVTVSS

SEQ ID NO: 13 - protein, 117 aa, Artificial Sequence
  Nanobody sequence
EVQLVESGGGSVQPGGSLRLSCAASGSVHKINFLGWYRQAPGKEREMVATITIGDATDYADSAKGRFTISRDEAKNMVYLQMNSLSPEDTAVYFCRAGSRLYPYNYWGQGTLVTVSS

SEQ ID NO: 14 - protein, 117 aa, Artificial Sequence
  Nanobody sequence
EVQLVESGGGLVQPGGSLRLSCAASGSVHLLNFLGWYRQAPGKEREMVAHISIADATDYAHFAKGRFTISRDEAKNMVYLQMNSLRPEDTAVYFCRAGSRIYPYDYWGRGTQVTVSS

SEQ ID NO: 15 - protein, 117 aa, Artificial Sequence
  Nanobody sequence
EVQLVESGGGLVQPGGSLRLSCRASGDVHKINILGWYRQAPAKEREMVAHITIGDATVYAESAKGRFTISRDEAKNMVYLQMNSLKPEDTAVYFCRAYSRIYPYNYWGQGTQVTVSS

SEQ ID NO: 16 - protein, 117 aa, Artificial Sequence
  Nanobody sequence
EVQLVESGGGLVQPGGSLRLSCAASGSVHLLNFLGWYRQCPGKEREMVAHITIADATDYSHFAKGRFTISRDEAKNMVYLQMNSLRPEDTAVYFCRAGSRIYPYDYWGQGTLVTVSS

SEQ ID NO: 17 - protein, 117 aa, Artificial Sequence
  Nanobody sequence
EVQLVESGGGLVQPGGSLRPSCAASGSVHLLNFLGWYRQAPGKEREMVAHITIADATDYAHFAKGRFTISRDEAKNMVYLQMNSLRPEDTAVYFCRAGSRIYPYDYWGQGTQVTVSS

SEQ ID NO: 18 - protein, 117 aa, Artificial Sequence
  Nanobody sequence
EVQLVESGGGLVQPGGSLRLSCAASGSVHLLNFLGWYRQAPGKEREMVAHITIADATDYAHFAKGRFTISRDEAKNMVYLQMNSLRPEDTAVYFCRAGSRIYPYDYWGQGTLVTVSS

SEQ ID NO: 19 - protein, 117 aa, Artificial Sequence
  Nanobody sequence
EVQLVESGGGLVQPGGSLKLSCAASGAVHKINFLGWYRQTPEKEREMVAHITIGDEVDYADSAKGRFTISRDEAKNMVYLQMTSLTPEDTAVYVCRAGSRLYPYNYWGQGTQVTVSS

SEQ ID NO: 20 - protein, 117 aa, Artificial Sequence
  Nanobody sequence
EVQLVESGGGLVHPGGSLRLSCAASGDVHKINFLGWHRQPPGKEREKVAHITIGDVTDYADSAKGRFTISRDEAKNMVYLQMNNLKPEDTAVYFCRAGSRIYPYDYWGQGTQVTVSS

SEQ ID NO: 21 - protein, 117 aa, Artificial Sequence
  Nanobody sequence
EVQLVESGGGLVQPGGSLRLSCAASGDVHKINVLGWYRQAPAKEREMVAHITIGDATDYADSAKGRFTISRDEAKNMVHLQMNSLKPEDTAVYFCRAYSRIYPYNYWGQGTQVTVSS

SEQ ID NO: 22 - protein, 117 aa, Artificial Sequence
  Nanobody sequence
EVQLVESGGGLVQPGGSLRLSCAASGDVHKINILGWYRQAPAKEREMVAHITIGDATNYADSAKGRFTISRDEAKNMVYLQMNSLKPEDTAVYFCRAYSRIYPYNYWGQGTLVTVSS

SEQ ID NO: 23 - protein, 117 aa, Artificial Sequence
  Nanobody sequence
EVQLVESGGGLVQPGGSLRLSCAASGDVHKINFLGWHRQAPGKEREKVAHITIGDVTDYADSAKGRFTISRDEAKNMVFLQMNNLKPEDTAVYFCRAGSRIYPYDYWGQGTQVTVSS

SEQ ID NO: 24 - protein, 117 aa, Artificial Sequence
  Nanobody sequence
EVQLVESGGGLVQPGGSLRLSCAASGDVHKINILGWYRQAPAKEREMVAHITIGDATDYAGSAKGRFTISRDEAKNMVYLQMNSLKPEDTAVYFCRAYSRIYPYNYWGQGTLVTVSS

SEQ ID NO: 25 - protein, 117 aa, Artificial Sequence
  Nanobody sequence
EVQLVESGGGLVQPGGSLRLSCAASGEVYKINFLGWYRQAPGKEREKVAHITIADVADYADFAKGRFTISRDEAKNMVYLQMNSLKPEDTAVYFCRAGSRIWPYDYWGQGTQVTVSS

SEQ ID NO: 26 - protein, 117 aa, Artificial Sequence
  Nanobody sequence
EVQLVESGGGLVQPGGSLKLSCAASGAVHKINFLGWYRQAPEKEREMVATITIGDEVDYADSAKGRFTISRDEAKNMVYLQMTSLKPEDTTVYVCRAGSRLYPYNYWGQGTQVTVSS

SEQ ID NO: 27 - protein, 117 aa, Artificial Sequence
  Nanobody sequence
EVQLVESGGGLVQPGGSLRLSCAASGEVYKINFLGWYRQAPGKEREKVAHITIADVADYADFAKGRFTISRDEAKNMVYLQMNSLKPEDTAVYFCRAGSRIWPYDYWGQGTLVTVSS

SEQ ID NO: 28 - protein, 117 aa, Artificial Sequence
  Nanobody sequence
EVQLVESGGGLVQPGGSLRLSCVASGDVHKINILGWYRQAPGKEREKVAHISISDQTDYAESAKGRFTISRDESKNMVYLQMNSLKPEDTAVYLCRAFSRIYPYDYWGQGTLVTVSS

SEQ ID NO: 29 - protein, 117 aa, Artificial Sequence
  Nanobody sequence
EVQLVESGGGLVQPGGSLRLSCAASGSVHKINFLGWYRQAPGKERELVATITIGDATDYADYAKGRFTISRDEARNMVYLQMNSLKPEDTAVYFCRAGSRLYPYNYWGQGTLVTVSS

SEQ ID NO: 30 - protein, 117 aa, Artificial Sequence
  Nanobody sequence
EVQLVESGGGLVQPGGSLRLSCAASGDVHKINILGWYRQAPAKEREMVAHITIGDATDYADSAKGRFAISRDEAKNMVYLQMNSLKPEDTAVYFCRAYSRIYPYNYWGQGTLVTVSS

SEQ ID NO: 31 - protein, 117 aa, Artificial Sequence
  Nanobody sequence
EVQLVESGGGLVQPGGSLRLSCAASGDVHKINFLGWHRQAPGKEREKVAHITIGDATDYADSAKGRFTISRDEAKNMVYLQMNSLKPEDTAVYFCRAGSRIYPYDYWGQGTQVTVSS

SEQ ID NO: 32 - protein, 117 aa, Artificial Sequence
  Nanobody sequence
EVQLVESGGGSVQPGGSLRLSCAASGSVHKINFLGWYRQAPGKEREVVATITIGDATDYADSAKGRFTISRDEAKNMVYLQMNSLSPEDTAVYFCRAGSRLYPYNYWGQGTQVTVSS

SEQ ID NO: 33 - protein, 117 aa, Artificial Sequence
  Nanobody sequence
EVQLVESGGGLVQPGGSARLSCVASGDVHKINFLGWYRQAPGKEREKVAHITIGDQTDYADSAKGRFTISRDEAKNMVYLQMNSLKPEDTAVYFCRAGSRIWPYDYWGQGTQVTVSS

SEQ ID NO: 34 - protein, 117 aa, Artificial Sequence
  Nanobody sequence
EVQLVESGGGLVQPGGSLRLSCAASGSVHLLNFLGWYRQAPGKEREMVAHITIADATDYSHFAKGRFTISRDEAKNMVYLQMNSLRPEDTAVYFCRAGSRIYPYDYWGQGTLVTVSS

SEQ ID NO: 35 - protein, 117 aa, Artificial Sequence
  Nanobody sequence
EVQLVESGGGLVQPGGSLRLSCAVSGSVHLLNFLGWYRQAPGKERGVVAHITIADATDYSHFAKGRFTISRDEAKNMVYLQMNSLRPEDTAVYFCRAGSRIYPYDYWGQGTQVTVSS

SEQ ID NO: 36 - protein, 117 aa, Artificial Sequence
  Nanobody sequence
EVQLVESGGGLVQAGGSLTLSCAASGDVHKINILGWYRQAPAKEREMVAHITIGDATDYADSAKGRFTISRDEAKNMVYLQMNSLKPEDTAVYFCRAYSRIYPYNYWGQGTLVTVSS

SEQ ID NO: 37 - protein, 117 aa, Artificial Sequence
  Nanobody sequence
EVQLVESGGGLVQPGGSLRLSCAASGGVHKINILGWYRQAPAKEREMVAHITIGDATDYADSAKGRFTISRDEAKNMVYLQMNSLKPEDTAVYFCRAYSRIYPYNYWGQGTLVTVSS

SEQ ID NO: 38 - protein, 117 aa, Artificial Sequence
  Nanobody sequence
EVQLVESGGGLVQPGGSLRLSCAASGEVYKINFLGWYRQAPGKEREKVAHITIADVADYADFAQGRFTISRDEAKNMVYLQMNSLKPEDTAVYFCRAGSRIWPYDYWGQGTQVTVSS

SEQ ID NO: 39 - protein, 117 aa, Artificial Sequence
  Nanobody sequence
EVQLVESGGGLVQPGGSLRLSCAASGDVHKINILGWYRQAPAKEREMVAHITIGDTTDYADSAKGRFTISRDEAKNMVYLQMNSLKPEDTAVYFCRAYSRIYPYNYWGQGTQVTVSS

SEQ ID NO: 40 - protein, 117 aa, Artificial Sequence
  Nanobody sequence
EVQLVESGGGLVQPGGSLRLSCAASGSVHLLNFLGWYRQAPGKEREMVAHITIADATDYSHFAKGRFTISRDEAKNMVYLQMNSLRPEDTAVYFCRAGSRIYPYDYWGHGTLVTVSS

SEQ ID NO: 41 - protein, 117 aa, Artificial Sequence
  Nanobody sequence
EVQLVESGGGLVQPGGSLRLSCVASGDVHKINFLGWYRQAPGKEREKVAHITIGDQADYADSAKGRFTISRDEAKNMVYLQMNSLKPEDTAVYFCRAGSRIYPYDYWGRGTLVTVSS

SEQ ID NO: 42 - protein, 117 aa, Artificial Sequence
  Nanobody sequence
EVQLVESGGGLVQPGGSLRLSCAVSGSVHLLNFLGWYRQAPGKEREMVTHITIADATDYSHFAKGRFTISRDEAKNMVYLQMNSLRPEDTAVYFCRAGSRIYPYDYWGQGTQVTVSS

SEQ ID NO: 43 - protein, 117 aa, Artificial Sequence
  Nanobody sequence
EVQLVESGGDLVQPGGSLRLSCAASGDVHKINFLGWYRQAPGKEREMVAHITIADATDYAEFAKGRFTISRDEPKNMVHLQMNSLKPEDTAVYLCRAGSRIYPYNYWGQGTQVTVSS

SEQ ID NO: 44 - protein, 117 aa, Artificial Sequence
  Nanobody sequence
EVQLVESGGGLVQPGGSLRLSCAASGDVHKINILGWYRQAPAKEREMVAHITIGDATDYADSAKGRFTISRDEAKNMVYLQMNSLKPEDTAVYFCRAYSRIYPYNYWGRGTQVTVSS

SEQ ID NO: 45 - protein, 117 aa, Artificial Sequence
  Nanobody sequence
EVQLVESGGGLVQPGGSLRLSCVASGDVHKINILGWYRQAPGKEREKVARISISDQTDYAESAKGRFTISRDESKNMVYLQMNSLKPEDTAVYLCRAFSRIYPYDYWGQGTLVTVSS

SEQ ID NO: 46 - protein, 117 aa, Artificial Sequence
  Nanobody sequence
EVQLVESGGGLVQPEGSLRLSCAASGEVYKINFLGWYRQAPGKEREKVAHITIADVADYADFAKGRLTISRDEAKNMVYLQMNSLKPEDTAVYFCRAGSRIWPYDYWGQGTLVTVSS

SEQ ID NO: 47 - protein, 117 aa, Artificial Sequence
  Nanobody sequence
EVQLVESGGGLVQPGGSLKLPCAASGAVHKINFLGWYRQTPEKEREMVATITIGDEVDYADSAKGRFTISRDEAKNMVYLQMTSLKPEDTAVYVCRAGSRLYPYNYWGQGTLVTVSS

SEQ ID NO: 48 - protein, 117 aa, Artificial Sequence
  Nanobody sequence
EVQLVESGGGLVQPGGSLGLSCAASGSVHLLNFLGWYRQAPGKEREMVAHITIADATDYAHFAKGRFTISRDEAKNMVYLQMNSLRPEDTAVYFCRAGSRIYPYDYWGQGTLVTVSS

SEQ ID NO: 49 - protein, 117 aa, Artificial Sequence
  Nanobody sequence
EVQLVESGGGLAQPGGSLRLSCAASGDVHKINILGWYRQAPAKEREMVAHITIGDATDYADSAKGRFTISRDEAKNMVYLQMNSLKPEDTAVYFCRAYSRIYPYNYWGQGTLVTVSS

SEQ ID NO: 50 - protein, 117 aa, Artificial Sequence
  Nanobody sequence
EVQLVESGGGLVQPGGSLRLSCVASGDVHKINFLGWYRQAPGKEREKVAHISIGDQTDYADSAKGRFTISRDESKNMVYLQMNSLKPEDTAVYFCRAFSRIYPYDYWGQGTLVTVSS

SEQ ID NO: 51 - protein, 117 aa, Artificial Sequence
  Nanobody sequence
EVQLVESGGGLVQPGGSLRLSCAASGEVYKINFLGWYRQAPGKEREKVAHITIADAADYADFAKGRFTISRDGAKNMVYLQMNSLKPEDTAVYFCRAGSRIWPYDYWGQGTQVTVSS

SEQ ID NO: 52 - protein, 117 aa, Artificial Sequence
  Nanobody sequence
EVQLVESGGGWVQPGGSLRLSCAASGSVYKINFLSWYRQAPGHERELVATITIGDAADYADSAKGRFTISRDEARNMVYLQMNSLKPEDTALYFCHAGSRLYPYNYWGQGTQVTVSS

SEQ ID NO: 53 - protein, 117 aa, Artificial Sequence
  Nanobody sequence
EVQLVESGGGLVQPGGSLRLSCAASGSVHLLNFLGWYRQAPGKEREMVAHITIADATDYSHFAKGRFTISRDEAKNMVYLQMNSLRPEDTAVYFCRAGSRIYPYDYWGQGTQVTVSS

SEQ ID NO: 54 - protein, 117 aa, Artificial Sequence
  Nanobody sequence
EVQLVESGGGLVQPGGSLRLSCVASGDVHKINILGWYRQAPGKEREKVAHIAISDQTDYAESAKGRFTISRDESKNMVYLQMNSLKPEDTAVYLCRAFSRIYPYDYWGQGTLVTVSS

SEQ ID NO: 55 - protein, 117 aa, Artificial Sequence
  Nanobody sequence
EVQLVESGGGLVQPGGSLRLSCAASGDVHKINILGWYRQAPAKEREMVAHITIGDATDYADSAKGRFTISRDEAKNMVYLQMNSLKPEDTAAYFCRAYSRIYPYNYWGQGTLVTVSS

SEQ ID NO: 56 - protein, 117 aa, Artificial Sequence
  Nanobody sequence
EVQLVESGGGLVQPGGSLRLSCAASGDVHKINILGWYRQAPAKERGMVAHITIGDATDYADSAKGRFTISRDEAKNMVYLQMNSLKPEDTAVYFCRAYSRIYPYNYWGQGTQVTVSS

SEQ ID NO: 57 - protein, 117 aa, Artificial Sequence
  Nanobody sequence
EVQLVESGGGLVQPGGSLRLSCAASGDVHKINILGWYRQAPAKEHEMVAHITIGDATDYADSAKGRFTISRDEAKNMVYLQMNSLKPEDTAVYFCRAYSRIYPYNYWGQGTLVTVSS

SEQ ID NO: 58 - protein, 117 aa, Artificial Sequence
  Nanobody sequence
EVQLVESGGGLVQPGGSLRLSCAASGDVHKINILGWYRQAPAREREMVAHITIGDATDYADSAKGRFTISRDEAKNMVYLQMNSLKPEDTAVYFCRAYSRIYPYNYWGQGTQVTVSS

SEQ ID NO: 59 - protein, 117 aa, Artificial Sequence
  Nanobody sequence
EVQLVESGGGLVQPGGSLRLSCAASGDVHKINILGWYRQAPAKEREMVAHITIGDATDYADSAKGRFTISRDEAENMVYLQMNSLKPEDTAVYFCRAYSRIYPYNYWGQGTLVTVSS

SEQ ID NO: 60 - protein, 117 aa, Artificial Sequence
  Nanobody sequence
EVQLVESGGGLVQPGGSLKLSCAASGAVHKINFLGWYRQTPEKEREMVATITIGDEVDYADSAKGRFTISRDEAKNMVYLQMTSLKPEDTAVYVCRAGSRLYPYNYWGQGTLVTVSS

SEQ ID NO: 61 - protein, 117 aa, Artificial Sequence
  Nanobody sequence
EVQLVESGGGLVQPGGSLKLSCAASGAVHKINFLGWYRQAPEKEREMVATITIGDEVDYADSAKGRFTISRDEATNMVYLQMTSLKPEDTAVYFCRAGSRIYPYNYWGQGTQVTVSS

SEQ ID NO: 62 - protein, 117 aa, Artificial Sequence
  Nanobody sequence
EVQLVESGGGLVQPGGSLRLSCAASGDVHKINILGWYRQAPAKEREMVAHITIGDATSYAGSAKGRFTISRDEAKNMVYLQLNNLKPEDTAVYFCRAYSRIYPYNYWGQGTLVTVSS

SEQ ID NO: 63 - protein, 117 aa, Artificial Sequence
  Nanobody sequence
EVQLVESGGGLVQPGGSLRLSCAASGDVHKINILGWYRQAPAKEREMVAHITIGDATSYADSAKGRFTISRDEAKNMVYLQLNNLKPEDTAVYFCRAYSRIYPYNYWGQGTLVTVSS

SEQ ID NO: 64 - protein, 117 aa, Artificial Sequence
  Nanobody sequence
EVQLVESGGDLVQPGGSLRLSCAASGDVHKINFLGWYRQAPGKEREMVAHITIADATDYAEFAKGRFTISRDEPKNMVYLQMNSLKPEDTAVYLCRAGSRIYPYNYWGQGTQVTVSS

SEQ ID NO: 65 - protein, 117 aa, Artificial Sequence
  Nanobody sequence
EVQLVESGGGLVQPGGSLKLSCAASGAVHKINFLGWYRQTPEKEREMVATITIGDEVDYAHSAKGRFTISRDEAKNMVYLQMTSLKPEDTAVYVCRAGSRLYPYNYWGQGTQVTVSS

SEQ ID NO: 66 - protein, 117 aa, Artificial Sequence
  Nanobody sequence
EVQLVESGGGLVQPGGSLKLSCAASGAVHKINFLGWYRQTPEKEREMVATITIGDEVAYADSAKGRFTISRDEAKNMVYLQMTSLKPEDTAVYVCRAGSRLYPYNYWGQGTQVTVSS

SEQ ID NO: 67 - protein, 117 aa, Artificial Sequence
  Nanobody sequence
EVQLVESGGGLVQPGGSLRLSCAASGEVYKINFLGWYRQAPGKEREKVAHITIADAADYADFAKGRFTISRDEAKNMVYLQMNSLKPEDTAVYFCRAGSRIWPYDYWGQGTQVTVSS

SEQ ID NO: 68 - protein, 117 aa, Artificial Sequence
  Nanobody sequence
EVQLVESGGGLVQPGGSLRLSCAASGEVYKINFLGWYRQAPGKEREKVAHITIADAADYADFAKGRFTISRDEAKNMVYLQMNSLKPEDTAVYFCRAGSRIYPYDYWGQGTQVTVSS

SEQ ID NO: 69 - protein, 117 aa, Artificial Sequence
  Nanobody sequence
EVQLVESGGGSVQPGGSLRPSCAASGSVHKINFLGWYRQAPGKEREMVATITIGDATDYADSAKGRFTISRDEAKNMVYLQMNSLSPEDTAVYFCRAGSRLYPYNYWGQGTQVTVSS

SEQ ID NO: 70 - protein, 117 aa, Artificial Sequence
  Nanobody sequence
EVQLVESGGGLVQPGGSLRLSCAASGEVYKINFLGWYRQAPGKEREKVAHITIADVADYADFAKGRFTISRDEVKNMVYLQMNSLKPEDTAVYFCRAGSRIWPYDYWGQGTLVTVSS

SEQ ID NO: 71 - protein, 117 aa, Artificial Sequence
  Nanobody sequence
EVQLVESGGGLVQPGESLRLSCAASGDVHKINILGWYRQAPAKEREMVAHITIGDATDYADSAKGRFTISRDEAKNMVYLQMNSLKPEDTAVYFCRAYSRIYPYNYWGQGTLVTVSS

SEQ ID NO: 72 - protein, 117 aa, Artificial Sequence
  Nanobody sequence
EVQLVESGGGLVQPGGSLRLSCAASGEVYKINFLGWYRQAPGKEREKVAHITIADAADYADFAKGRFTISRDEAKNMVYLQMNSLRPEDTAVYFCRAGSRIWPYDYWGQGTQVTVSS

SEQ ID NO: 73 - protein, 117 aa, Artificial Sequence
  Nanobody sequence
EVQLVESGGGLVQPGGSLRLSCAASGSVHLLNFLGWYRQAPGKEREMVAHITIADVTDYSYFAKGRFTISRDEAKNMVYLQMNSLRPEDTAVYFCRAGSRIYPYDYWGQGTQVTVSS

SEQ ID NO: 74 - protein, 117 aa, Artificial Sequence
  Nanobody sequence
EVQLVESGGGLVQPGGSLRLSCAASGDVHKINILGWYRQAPAKEREMVAHITIGDATDYADSAKGRFTISRDEAKNVVYLQMNSLKPEDTAVYFCRAYSRIYPYNYWGQGTLVTVSS

SEQ ID NO: 75 - protein, 117 aa, Artificial Sequence
  Nanobody sequence
EVQLVESGGGSVQPGGSLRLSCAASGSVHKINFLGWYRQAPGKERGMVATITIGDATDYADSAKGRFTISRDEAKNMVYLQMNSLSPEDTAVYFCRAGSRLYPYNYWGQGTQVTVSS

SEQ ID NO: 76 - protein, 117 aa, Artificial Sequence
  Nanobody sequence
EVQLVESGGGLVQPGGSLKLSCAASGAVHKINFLGWYRQTPEKEREMVATITIGDEVDYEDSAKGRFTISRDEAKNMVYLQMTGLKPEDTAVYVCRAGSRLYPYNYWGQGTLVTVSS

SEQ ID NO: 77 - protein, 117 aa, Artificial Sequence
  Nanobody sequence
EVQLVESGGGLVRPGGSLRLSCVASGDVHKINILGWYRQAPGKEREKVAHISISDQTDYAESAKGRFTISRDESKNMVYLQMNSLKPEDTAVYLCRAFSRIYPYDYWGQGTQVTVSS

SEQ ID NO: 78 - protein, 117 aa, Artificial Sequence
  Nanobody sequence
EVQLVESGGGLVQPGGSLRLSCAASGDVYKINFLGWHRQAPGKEREKVAHITIGDATDYADSAKGRFTISRDEAKNMVYLQMNSLKPEDTAVYFCRAGSRIYPYDYWGQGTLVTVSS

SEQ ID NO: 79 - protein, 117 aa, Artificial Sequence
  Nanobody sequence
EVQLVESGGGLVQPGGSLRLSCRASGDVHKINILGWYRQAPAKEREMIAHITIGDATDYAESAKGRFTISRDEAKNMVYLQMNSLKPEDTAVYFCRAYSRIYPYNYWGQGTQVTVSS

SEQ ID NO: 80 - protein, 117 aa, Artificial Sequence
  Nanobody sequence
EVQLVESGGGLVQPGGSLRLSCAASGDVHKINILGWYRQAPAKGREMVAHITIGDATDYADSAKGRFTISRDEAKNMVYLQMNSLKPEDTAVYFCRAYSRIYPYNYWGQGTQVTVSS

SEQ ID NO: 81 - protein, 117 aa, Artificial Sequence
  Nanobody sequence
EVQLVESGGDLVQPGGSLRLSCAASGDVHKINFLGWYRQAPGKEREMVAHITIADATDYAEFAKGRFTISRDEPKNMVYLQMNSLKPEDTAVYLCRAGSRIYPYSYWGQGTQVTVSS

SEQ ID NO: 82 - protein, 117 aa, Artificial Sequence
  Nanobody sequence
EVQLVESGGGMVQPGGSLRLSCAASGDVHKINILGWYRQAPAKEREMVAHITIGDATDYADSAKGRFTISRDEAKNMVYLQMNSLKPEDTAVYFCRAYSRIYPYNYWGQGTLVTVSS

SEQ ID NO: 83 - protein, 117 aa, Artificial Sequence
  Nanobody sequence
EVQLVESGGGLVQPGGSLRLSCAASGDVHKINILGWYRQVPAKEREMVAHITIGDATDYADSAKGRFTISRDEAKNMVYLQMNSLKPEDTAAYFCRAYSRIYPYNYWGQGTLVTVSS

SEQ ID NO: 84 - protein, 117 aa, Artificial Sequence
  Nanobody sequence
EVQLVESGGGLVQPGGSLRLSCAASGEVYKINFLGWYRQAPGKEREKVAHITIADAADYADFAKGRFTISRDEAKNMVYLQMNSLKPEDTAVYFCRAGSRIWPYDYWGQGTLVTVSS

SEQ ID NO: 85 - protein, 117 aa, Artificial Sequence
  Nanobody sequence
EVQLVESGGGLVQPGGSLRLSCAASGSVHLLNFLGWYRQAPGKEREMVAHITIADATDYSHFAKGRFTISRDEAKNMVYLQMNGLRPEDTAVYFCRAGSRIYPYDYWGQGTLVTVSS

SEQ ID NO: 86 - protein, 117 aa, Artificial Sequence
  Nanobody sequence
EVQLVESGGGLVQPGGSLRLSCAASGDVHKINFLGWYRQAPGKEREMVAHITIADATDYAEFAKGRFTISRDEPKNMVYLQMNSLKPEDTAVYLCRAGSRIYPYNYWGQGTQVTVSS

SEQ ID NO: 87 - protein, 117 aa, Artificial Sequence
  Nanobody sequence
EVQLVESGGGLVQPGGSLRLSCAASGEVHKINILGWYRQCPGKERDMVATITIGDATDYADSAKGRFTISRDEAKNMVYLQMNSLKPEDTAVYFCRALSRLYPYNYWGQGTLVTVSS

SEQ ID NO: 88 - protein, 117 aa, Artificial Sequence
  Nanobody sequence
EVQLVESGGGLVQPGGSLRLSCAASGDVHKINILGWYRQAPAKEREMVAHITIGDATDYADSAKGRFTISRDEAKNMVYLQMNSLKPEDTAVYLCRAYSRIYPYNYWGQGTQVTVSS

SEQ ID NO: 89 - protein, 117 aa, Artificial Sequence
  Nanobody sequence
EVQLVESGGGLVQPGGSLRLSCAASGEVYKINFLGWQRQAPGKEREKVAHITIADVADYADFAKGRFTISRDEAKNMVYLQMNSLKPEDTAVYFCRAGSRIWPYDYWGQGTLVTVSS

SEQ ID NO: 90 - protein, 117 aa, Artificial Sequence
  Nanobody sequence
EVQLVESGGDLVQPGGSLRLSCAASGDVHKINFLGWYRQAPGKEREMVAHITIADATDYAEFAKGRFTISRDEPKNMVYLQMNSLKPVDTAVYLCRAGSRIYPYNYWGQGTLVTVSS

SEQ ID NO: 91 - protein, 117 aa, Artificial Sequence
  Nanobody sequence
EVQLVESGGGLVQPGGSLRLSCAASGSVHLLNFLGWYRQAPGKEREKVAHITIADATDYSHFAKGRFTISRDEAKNMVYLQMNNLRPEDTAVYFCRAGSRIYPYDYWGQGTLVTVSS

SEQ ID NO: 92 - protein, 117 aa, Artificial Sequence
  Nanobody sequence
EVQLVESGGGLVQPGGSPRLSCVASGDVHKINFLGWYRQAPGKEREKVAHITIGDQADYADSAKGRFTISRDEAKNMVYLQMNSLKPEDTAVYFCRAGSRIYPYDYWGQGTLVTVSS

SEQ ID NO: 93 - protein, 117 aa, Artificial Sequence
  Nanobody sequence
EVQLVESGGGLVQPGGSLRLSCAASGDVHKINILGWYRQAPAKEREMVAHITIGDATDYADSAKGRFTISRDEAKNMVYLQMNSLKPEDAAVYFCRAYSRIYPYNYWGQGTLVTVSS

SEQ ID NO: 94 - protein, 117 aa, Artificial Sequence
  Nanobody sequence
EVQLVESGGGLVQPGGSLRLSCAASGEVYKINFLGWYRQAPGKEREKVAHITIADVADYADFAKGRFTISRDGAKNMVYLQMNSLKPEDTAVYFCRAGSRIWPYDYWGQGTLVTVSS

SEQ ID NO: 95 - protein, 117 aa, Artificial Sequence
  Nanobody sequence
EVQLVESGGGSVQPGGSLRLSCAASGSVHKINFLGWYCQAPGKEREMVATITIGDATDYADSAKGRFTISRDEAKNMVYLQMNSLSPEDTAVYFCRAGSRLYPYNYWGQGTQVTVSS

SEQ ID NO: 96 - protein, 117 aa, Artificial Sequence
  Nanobody sequence
EVQLVESGGGLVQPGGSLRLSCVASGDVHKINILGWYRQAPGKEREKVAHISISDQTDYAESAKGRFTISRDESKNMVYLQMNSLKPEDAAVYLCRAFSRIYPYDYWGQGTQVTVSS

SEQ ID NO: 97 - protein, 117 aa, Artificial Sequence
  Nanobody sequence
EVQLVESGGGLVQPGGSLRPSCAASGEVYKINFLGWYRQAPGKEREKVAHITIADVADYADFAKGRFTISRDEAKNMVYLQMNSLKPEDTAVYFCRAGSRIWPYDYWGQGTQVTVSS

SEQ ID NO: 98 - protein, 117 aa, Artificial Sequence
  Nanobody sequence
EVQLVESGGGLVQPGGSLRPSCVASGDVHKINFLGWYRQAPGKEREKVAHITIADQADYADSAKGRFTISRDEAKNMVYLQMNSLKPEDTAVYFCRAGSRIYPYDYWGQGTLVTVSS

SEQ ID NO: 99 - protein, 117 aa, Artificial Sequence
  Nanobody sequence
EVQLVESGGGLVQPGGSLRLSCAASGEVHKINILGWYRQAPGKERDMVATITIGDETQYADSAKGRFTISRDEAKNMVYLQMNSLKPEDTAVYFCRALSRLYPYNYWGQGTLVTVSS

SEQ ID NO: 100 - protein, 117 aa, Artificial Sequence
  Nanobody sequence
EVQLVESGGGLVQPGGSLRLSCAASGDVHKINILGWYRQAPAKEREMVAHITIGDATDYADSAKGRFTISRDEAKNMVYLQMDSLKPEDTAVYFCRAYSRIYPYNYWGQGTLVTVSS

SEQ ID NO: 101 - protein, 117 aa, Artificial Sequence
  Nanobody sequence
EVQLVESGGGLVQPGGSLRLSCAASGDVHKINILGWYRQAPAKEREMVAHITIGDATDYADSAKGRFTISRDEAKNMVYLQMNSLKPGDTAVYFCRAYSRIYPYNYWGQGTLVTVSS

SEQ ID NO: 102 - protein, 117 aa, Artificial Sequence
  Nanobody sequence
EVQLVESGGGLVQPGGSLRLSCAASGDVHKINILGWHRQAPAKEREMVAHITIGDATDYADSAKGRFTISRDEAKNMVYLQMNSLKPEDTAVYFCRAYSRIYPYNYWGQGTLVTVSS

SEQ ID NO: 103 - protein, 117 aa, Artificial Sequence
  Nanobody sequence
EVQLVESGGGLVQPGGSLRLSCAASGDVHKINILGWHRQAPAKEREMVAHITIGDATDYADSAKGRFTISRDEAKNMVYLQMNSLKPEDTAAYFCRAYSRIYPYNYWGQGTQVTVSS

SEQ ID NO: 104 - protein, 117 aa, Artificial Sequence
  Nanobody sequence
EVQLVESGGGWVQAGGSLRLSCAASGDVHKINILGWYRQAPAKEREMVAHITIGDATDYADSAKGRFTISRDEAKNMVYLQMNSLKPEDTAVYFCRAYSRIYPYNYWGQGTLVTVSS

SEQ ID NO: 105 - protein, 117 aa, Artificial Sequence
  Nanobody sequence
EVQLVESGGGLVQPGGSLRLSCITSGETFKINIWGWYRQAPGKQRELVASLTIGGATDYADSVKGRFTISEDSAKNTVYLQMNSLKAEDTAVYFCNAKSRLYPYDYWGQGTQVTVSS

SEQ ID NO: 106 - protein, 117 aa, Artificial Sequence
  Nanobody sequence
EVQLVESGGGLVQPGGSLRLSCITSGETFKINIWGWYRQAPGKQRELVASLTIGGATNYADSVKGRFTISEDSAKNTVYLQMNSLKPEDTAVYFCNAKSRLYPYDYWGQGTLVTVSS

SEQ ID NO: 107 - protein, 117 aa, Artificial Sequence
  Nanobody sequence
EVQLVESGGGLVQPGGSLRLSCITSGETFKINIWGWYRQAPGKRRELVASLTIGGATNYADSVKGRFTISEDSAKNTVYLQMNSLKPEDTAVYFCNAKSRIYPYDYWGQGTQVTVSS

SEQ ID NO: 108 - protein, 117 aa, Artificial Sequence
  Nanobody sequence
EVQLVESGGGLVQPGGSLRLSCITSGETFKINIWGWYRQTPGKQRELVASLTIGGATNYADSVKGRFTISEDSAKNTVYLQMNSLKPEDTAVYFCNAKSRLYPYDYWGQGTQVTVSS

SEQ ID NO: 109 - protein, 117 aa, Artificial Sequence
  Nanobody sequence
EVQLVESGGGLVQPGGSLRLSCITSGQTFKINIWGWYRQAPGKQRELVASLTIGGATNYADSVKGRFTISEDSAKNTVYLQMNSLKPEDTAVYFCNAKSRLYPYDYWGQGTQVTVSS

SEQ ID NO: 110 - protein, 117 aa, Artificial Sequence
  Nanobody sequence
EVQLVESGGGLVQPGGSLRLSCITSGETFKVNIWGWYRQGPGKQRELVASLTIGGATNYADSVKGRFTISEDSAKNTVYLQMNSLKPEDTAVYFCNAKSRLYPYDYWGRGTQVTVSS

SEQ ID NO: 111 - protein, 118 aa, Artificial Sequence
  Nanobody sequence
EVQLVEESGGGLVQPGGSLRLSCITSGETFKINIWGWYRQAPGKQRELVASLTIGGATNYADSVKGRFTISEDSAKNTVYLQMNSLKPEDTAVYFCNAKSRIYPYDYWGRGTQVTVSS

SEQ ID NO: 112 - protein, 117 aa, Artificial Sequence
  Nanobody sequence
EVQLVESGGGLVQPGGSLRLSCITSGETFKINIWGWYRQAPGKQRELVASLTIGGATNYADSVKGRFTISEDSAKNTVYLQMNSLKPEDTAVYFCNAKSRLYPYDYWDQGTQVTVSS

SEQ ID NO: 113 - protein, 117 aa, Artificial Sequence
  Nanobody sequence
EVQLVESGGGLVQPGGSLRLSCLTSGETFKVNIWGWYRQGPGKQRELVASLTIGGATNYADSVKGRFTISEDSAKNTVYLQMSSLKPEDTAVYFCNAKSRLYPYDYWGQGTQVTVSS

SEQ ID NO: 114 - protein, 117 aa, Artificial Sequence
  Nanobody sequence
EVQLVESGGGLVQPGGSLRLSCITSGETFKINIWGWYRQAPGKQRELVASLTIGGATNYADSVKGRFTISEDSAKNTVYLQMNSLKPEDTAVYFCNAKSRIYPYDYWGRGTQVTVSS

SEQ ID NO: 115 - protein, 117 aa, Artificial Sequence
  Nanobody sequence
EVQLVESGGGLVQPGGSLRLSCITSGETFKINIWGWYRQAPGKQRELVASLTIGGATNYADSVKGRFTISEDSAKDTVYLQMNSLKPEDTAVYFCNAKSRLYPYDYWGQGTLVTVSS

SEQ ID NO: 116 - protein, 117 aa, Artificial Sequence
  Nanobody sequence
EVQLVESGGGLVQPGGSLRLSCAASGEIGRINFYRWYRQAPGNQREVVATITIADKTDYADSAKGRFTISRDESRNMVYLQMSSLKPEDTAVYFCHAGSRLYPYDYWGQGTQVTVSS

SEQ ID NO: 117 - protein, 117 aa, Artificial Sequence
  Nanobody sequence
EVQLVESGGGLVQPGGSLRLSCAASGEIGRINFYRWYRQAPGNQRGVVATITIADKIDYADSAKGRFTISRDESRNMVYLQMGSLKPEDTAVYFCHAGSRLYPYDYWGQGTQVTVSS

SEQ ID NO: 118 - protein, 117 aa, Artificial Sequence
  Nanobody sequence
EVQLVESGGGLVQPGGSLRLSCAASGEIGRINFYRWYRQAPGNQREVVATITIADKTDYADSAKGRFTISRDESRNMVYLQMSSLKPENTAVYFCHAGSRLYPYDYWGQGTQVTVSS

SEQ ID NO: 119 - protein, 10 aa, Artificial Sequence
  CDR1
GSVHKINFLG

SEQ ID NO: 120 - protein, 10 aa, Artificial Sequence
  CDR1
GSVHLLNFLG

SEQ ID NO: 121 - protein, 10 aa, Artificial Sequence
  CDR1
GAVHKINFLG

SEQ ID NO: 122 - protein, 10 aa, Artificial Sequence
  CDR1
GDVHKINILG

SEQ ID NO: 123 - protein, 10 aa, Artificial Sequence
  CDR1
GDVHKINFLG

SEQ ID NO: 124 - protein, 10 aa, Artificial Sequence
  CDR1
GETFKINIWG

SEQ ID NO: 125 - protein, 10 aa, Artificial Sequence
  CDR1
GDVHKINVLG

SEQ ID NO: 126 - protein, 10 aa, Artificial Sequence
  CDR1
GEVYKINFLG

SEQ ID NO: 127 - protein, 10 aa, Artificial Sequence
  CDR1
GGVHKINILG

SEQ ID NO: 128 - protein, 10 aa, Artificial Sequence
  CDR1
GQTFKINIWG

SEQ ID NO: 129 - protein, 10 aa, Artificial Sequence
  CDR1
GSVYKINFLS

SEQ ID NO: 130 - protein, 10 aa, Artificial Sequence
  CDR1
GEIGRINFYR

SEQ ID NO: 131 - protein, 10 aa, Artificial Sequence
  CDR1
GETFKVNIWG

SEQ ID NO: 132 - protein, 10 aa, Artificial Sequence
  CDR1
GDVYKINFLG

SEQ ID NO: 133 - protein, 10 aa, Artificial Sequence
  CDR1
GEVHKINILG

SEQ ID NO: 134 - protein, 9 aa, Artificial Sequence
  CDR2
TITIGDTTD

SEQ ID NO: 135 - protein, 9 aa, Artificial Sequence
  CDR2
TITIGDATD

SEQ ID NO: 136 - protein, 9 aa, Artificial Sequence
  CDR2
HITIADATD

SEQ ID NO: 137 - protein, 9 aa, Artificial Sequence
  CDR2
TITIGDDVD

SEQ ID NO: 138 - protein, 9 aa, Artificial Sequence
  CDR2
HITIGDATD

SEQ ID NO: 139 - protein, 9 aa, Artificial Sequence
  CDR2
HITIGDQAD

SEQ ID NO: 140 - protein, 9 aa, Artificial Sequence
  CDR2
HISIADATD

SEQ ID NO: 141 - protein, 9 aa, Artificial Sequence
  CDR2
HITIGDATV

SEQ ID NO: 142 - protein, 9 aa, Artificial Sequence
  CDR2
SLTIGGATD

SEQ ID NO: 143 - protein, 9 aa, Artificial Sequence
  CDR2
HITIGDEVD

SEQ ID NO: 144 - protein, 9 aa, Artificial Sequence
  CDR2
HITIGDVTD

SEQ ID NO: 145 - protein, 9 aa, Artificial Sequence
  CDR2
SLTIGGATN

SEQ ID NO: 146 - protein, 9 aa, Artificial Sequence
  CDR2
HITIGDATN

SEQ ID NO: 147 - protein, 9 aa, Artificial Sequence
  CDR2
HITIADVAD

SEQ ID NO: 148 - protein, 9 aa, Artificial Sequence
  CDR2
TITIGDEVD

SEQ ID NO: 149 - protein, 9 aa, Artificial Sequence
  CDR2
HISISDQTD

SEQ ID NO: 150 - protein, 9 aa, Artificial Sequence
  CDR2
HITIGDQTD

SEQ ID NO: 151 - protein, 9 aa, Artificial Sequence
  CDR2
HITIGDTTD

SEQ ID NO: 152 - protein, 9 aa, Artificial Sequence
  CDR2
RISISDQTD

SEQ ID NO: 153 - protein, 9 aa, Artificial Sequence
  CDR2
HISIGDQTD

SEQ ID NO: 154 - protein, 9 aa, Artificial Sequence
  CDR2
HITIADAAD

SEQ ID NO: 155 - protein, 9 aa, Artificial Sequence
  CDR2
TITIGDAAD

SEQ ID NO: 156 - protein, 9 aa, Artificial Sequence
  CDR2
HIAISDQTD

SEQ ID NO: 157 - protein, 9 aa, Artificial Sequence
  CDR2
TITIADKTD

SEQ ID NO: 158 - protein, 9 aa, Artificial Sequence
  CDR2
TITIADKID

SEQ ID NO: 159 - protein, 9 aa, Artificial Sequence
  CDR2
HITIGDATS

SEQ ID NO: 160 - protein, 9 aa, Artificial Sequence
  CDR2
TITIGDEVA

SEQ ID NO: 161 - protein, 9 aa, Artificial Sequence
  CDR2
HITIADVTD

SEQ ID NO: 162 - protein, 9 aa, Artificial Sequence
  CDR2
HITIADQAD

SEQ ID NO: 163 - protein, 9 aa, Artificial Sequence
  CDR2
TITIGDETQ

SEQ ID NO: 164 - protein, 9 aa, Artificial Sequence
  CDR3
GSRLYPYNY

SEQ ID NO: 165 - protein, 9 aa, Artificial Sequence
  CDR3
GSRIYPYDY

SEQ ID NO: 166 - protein, 9 aa, Artificial Sequence
  CDR3
YSRIYPYNY

SEQ ID NO: 167 - protein, 9 aa, Artificial Sequence
  CDR3
KSRLYPYDY

SEQ ID NO: 168 - protein, 9 aa, Artificial Sequence
  CDR3
KSRIYPYDY

SEQ ID NO: 169 - protein, 9 aa, Artificial Sequence
  CDR3
GSRIWPYDY

SEQ ID NO: 170 - protein, 9 aa, Artificial Sequence
  CDR3
FSRIYPYDY

SEQ ID NO: 171 - protein, 9 aa, Artificial Sequence
  CDR3
GSRIYPYNY

SEQ ID NO: 172 - protein, 9 aa, Artificial Sequence
  CDR3
GSRLYPYDY

SEQ ID NO: 173 - protein, 9 aa, Artificial Sequence
  CDR3
GSRIYPYSY

SEQ ID NO: 174 - protein, 9 aa, Artificial Sequence
  CDR3
LSRLYPYNY

SEQ ID NO: 175 - protein, 25 aa, Artificial Sequence [sequence omitted]

SEQ ID NO: 176 - protein, 25 aa, Artificial Sequence
  FR1
EVQLVESGGGLVQPGRSLRLPCAAS

SEQ ID NO: 177 - protein, 25 aa, Artificial Sequence [sequence omitted]

SEQ ID NO: 178 - protein, 25 aa, Artificial Sequence
  FR1
EVQLVESGGGLVQPGGSLKLSCAAS

SEQ ID NO: 179 - protein, 25 aa, Artificial Sequence
  FR1
EVQLVESGGGLVQPGGSLRLSCRAS

SEQ ID NO: 180 - protein, 25 aa, Artificial Sequence
  FR1
EVQLVESGGGLVRPGGSLRLSCAAS

SEQ ID NO: 181 - protein, 25 aa, Artificial Sequence
  FR1
EVQLVESGGGLVQPGGSLRLSCVAS

SEQ ID NO: 182 - protein, 25 aa, Artificial Sequence
  FR1
EVQLVESGGGSVQPGGSLRLSCAAS

SEQ ID NO: 183 - protein, 25 aa, Artificial Sequence
  FR1
EVQLVESGGGLVQPGGSLRPSCAAS

SEQ ID NO: 184 - protein, 25 aa, Artificial Sequence
  FR1
EVQLVESGGGLVQPGGSLRLSCITS

SEQ ID NO: 185 - protein, 25 aa, Artificial Sequence
  FR1
EVQLVESGGGLVHPGGSLRLSCAAS

SEQ ID NO: 186 - protein, 25 aa, Artificial Sequence
  FR1
EVQLVESGGGLVQPGGSARLSCVAS

SEQ ID NO: 187 - protein, 25 aa, Artificial Sequence
  FR1
EVQLVESGGGLVQAGGSLTLSCAAS

SEQ ID NO: 188 - protein, 25 aa, Artificial Sequence
  FR1
EVQLVESGGDLVQPGGSLRLSCAAS

SEQ ID NO: 189 - protein, 25 aa, Artificial Sequence
  FR1
EVQLVESGGGLVQPEGSLRLSCAAS

SEQ ID NO: 190 - protein, 25 aa, Artificial Sequence
  FR1
EVQLVESGGGLVQPGGSLKLPCAAS

SEQ ID NO: 191 - protein, 25 aa, Artificial Sequence
  FR1
EVQLVESGGGLVQPGGSLGLSCAAS

SEQ ID NO: 192 - protein, 25 aa, Artificial Sequence
  FR1
EVQLVESGGGLAQPGGSLRLSCAAS

SEQ ID NO: 193 - protein, 25 aa, Artificial Sequence
  FR1
EVQLVESGGGWVQPGGSLRLSCAAS

SEQ ID NO: 194 - protein, 25 aa, Artificial Sequence
  FR1
EVQLVESGGGSVQPGGSLRPSCAAS

SEQ ID NO: 195 - protein, 25 aa, Artificial Sequence
  FR1
EVQLVESGGGLVQPGESLRLSCAAS

SEQ ID NO: 196 - protein, 26 aa, Artificial Sequence
  FR1
EVQLVEESGGGLVQPGGSLRLSCITS

SEQ ID NO: 197 - protein, 25 aa, Artificial Sequence
  FR1
EVQLVESGGGLVRPGGSLRLSCVAS

SEQ ID NO: 198 - protein, 25 aa, Artificial Sequence
  FR1
EVQLVESGGGMVQPGGSLRLSCAAS

SEQ ID NO: 199 - protein, 25 aa, Artificial Sequence
  FR1
EVQLVESGGGLVQPGGSLRLSCLTS

SEQ ID NO: 200 - protein, 25 aa, Artificial Sequence
  FR1
EVQLVESGGGLVQPGGSPRLSCVAS

SEQ ID NO: 201 - protein, 25 aa, Artificial Sequence
  FR1
EVQLVESGGGLVQPGGSLRPSCVAS

SEQ ID NO: 202 - protein, 25 aa, Artificial Sequence
  FR1
EVQLVESGGGWVQAGGSLRLSCAAS

SEQ ID NO: 203 - protein, 14 aa, Artificial Sequence
  FR2
WYRQAPGKERELVA

SEQ ID NO: 204 - protein, 14 aa, Artificial Sequence
  FR2
WYRQAPGKERGLVA

SEQ ID NO: 205 - protein, 14 aa, Artificial Sequence
  FR2
WYRQAPGKEREMVA

SEQ ID NO: 206 - protein, 14 aa, Artificial Sequence
  FR2
WYRQTPEKEREMVA

SEQ ID NO: 207 - protein, 14 aa, Artificial Sequence
  FR2
WYRQAPAKEREMVA

SEQ ID NO: 208 - protein, 14 aa, Artificial Sequence
  FR2
WYRQAPGKEREKVA

SEQ ID NO: 209 - protein, 14 aa, Artificial Sequence
  FR2
WYRQCPGKEREMVA

SEQ ID NO: 210 - protein, 14 aa, Artificial Sequence
  FR2
WYRQAPGKQRELVA

SEQ ID NO: 211 - protein, 14 aa, Artificial Sequence
  FR2
WHRQPPGKEREKVA

SEQ ID NO: 212 - protein, 14 aa, Artificial Sequence
  FR2
WYRQAPGKRRELVA

SEQ ID NO: 213 - protein, 14 aa, Artificial Sequence
  FR2
WHRQAPGKEREKVA

SEQ ID NO: 214 - protein, 14 aa, Artificial Sequence
  FR2
WYRQAPEKEREMVA

SEQ ID NO: 215 - protein, 14 aa, Artificial Sequence
  FR2
WYRQAPGKEREVVA

SEQ ID NO: 216 - protein, 14 aa, Artificial Sequence
  FR2
WYRQAPGKERGVVA

SEQ ID NO: 217 - protein, 14 aa, Artificial Sequence
  FR2
WYRQTPGKQRELVA

SEQ ID NO: 218 - protein, 14 aa, Artificial Sequence
  FR2
WYRQAPGKEREMVT

SEQ ID NO: 219 - protein, 14 aa, Artificial Sequence
  FR2
WYRQAPGHERELVA

SEQ ID NO: 220 - protein, 14 aa, Artificial Sequence
  FR2
WYRQAPGNQREVVA

SEQ ID NO: 221 - protein, 14 aa, Artificial Sequence
  FR2
WYRQAPGNQRGVVA

SEQ ID NO: 222 - protein, 14 aa, Artificial Sequence
  FR2
WYRQAPAKERGMVA

SEQ ID NO: 223 - protein, 14 aa, Artificial Sequence
  FR2
WYRQAPAKEHEMVA

SEQ ID NO: 224 - protein, 14 aa, Artificial Sequence
  FR2
WYRQAPAREREMVA

SEQ ID NO: 225 - protein, 14 aa, Artificial Sequence
  FR2
WYRQGPGKQRELVA

SEQ ID NO: 226 - protein, 14 aa, Artificial Sequence
  FR2
WYRQAPGKERGMVA

SEQ ID NO: 227 - protein, 14 aa, Artificial Sequence
  FR2
WYRQAPAKEREMIA

SEQ ID NO: 228 - protein, 14 aa, Artificial Sequence
  FR2
WYRQAPAKGREMVA

SEQ ID NO: 229 - protein, 14 aa, Artificial Sequence
  FR2
WYRQVPAKEREMVA

SEQ ID NO: 230 - protein, 14 aa, Artificial Sequence
  FR2
WYRQCPGKERDMVA

SEQ ID NO: 231 - protein, 14 aa, Artificial Sequence
  FR2
WQRQAPGKEREKVA

SEQ ID NO: 232 - protein, 14 aa, Artificial Sequence
  FR2
WYCQAPGKEREMVA

SEQ ID NO: 233 - protein, 14 aa, Artificial Sequence
  FR2
WYRQAPGKERDMVA

SEQ ID NO: 234 - protein, 14 aa, Artificial Sequence
  FR2
WHRQAPAKEREMVA

SEQ ID NO: 235 - protein, 39 aa, Artificial Sequence
  FR3
YADSAKGRFTISRDEAKNMVYLQMNSLKPEDTAVHFCRA

SEQ ID NO: 236 - protein, 39 aa, Artificial Sequence
  FR3
YADYAKGRFTISRDEARNMVYLQMNSLKPEDTAVYFCRA

SEQ ID NO: 237 - protein, 39 aa, Artificial Sequence
  FR3
YADSAKGRFTISRDEAKNMVYLQMNSLKPEDTAVYFCRA

SEQ ID NO: 238 - protein, 39 aa, Artificial Sequence
  FR3
YSHFAKGRFTISRDEAKNMVYLQMNSLRPEDTAVYFCRA

SEQ ID NO: 239 - protein, 39 aa, Artificial Sequence
  FR3
YADSAKGRFTISRDEAKNMVYLQMTSLKPEDTAVYVCRA

SEQ ID NO: 240 - protein, 39 aa, Artificial Sequence
  FR3
YAESAKGRFTISRDEAKNMVYLQMNSLKPEDTAVYFCRA

SEQ ID NO: 241 - protein, 39 aa, Artificial Sequence
  FR3
YADSAKGRFTISRDEAKNMVYLQMNSLSPEDTAVYFCRA

SEQ ID NO: 242 - protein, 39 aa, Artificial Sequence
  FR3
YAHFAKGRFTISRDEAKNMVYLQMNSLRPEDTAVYFCRA

SEQ ID NO: 243 - protein, 39 aa, Artificial Sequence
  FR3
YADSVKGRFTISEDSAKNTVYLQMNSLKAEDTAVYFCNA

SEQ ID NO: 244 - protein, 39 aa, Artificial Sequence
  FR3
YADSAKGRFTISRDEAKNMVYLQMTSLTPEDTAVYVCRA

SEQ ID NO: 245 - protein, 39 aa, Artificial Sequence
  FR3
YADSAKGRFTISRDEAKNMVYLQMNNLKPEDTAVYFCRA

SEQ ID NO: 246 - protein, 39 aa, Artificial Sequence
  FR3
YADSVKGRFTISEDSAKNTVYLQMNSLKPEDTAVYFCNA

SEQ ID NO: 247 - protein, 39 aa, Artificial Sequence
  FR3
YADSAKGRFTISRDEAKNMVHLQMNSLKPEDTAVYFCRA

SEQ ID NO: 248 - protein, 39 aa, Artificial Sequence
  FR3
YADSAKGRFTISRDEAKNMVFLQMNNLKPEDTAVYFCRA

SEQ ID NO: 249 - protein, 39 aa, Artificial Sequence
  FR3
YAGSAKGRFTISRDEAKNMVYLQMNSLKPEDTAVYFCRA

SEQ ID NO: 250 - protein, 39 aa, Artificial Sequence
  FR3
YADFAKGRFTISRDEAKNMVYLQMNSLKPEDTAVYFCRA

SEQ ID NO: 251 - protein, 39 aa, Artificial Sequence
  FR3
YADSAKGRFTISRDEAKNMVYLQMTSLKPEDTTVYVCRA

SEQ ID NO: 252 - protein, 39 aa, Artificial Sequence
  FR3
YAESAKGRFTISRDESKNMVYLQMNSLKPEDTAVYLCRA

SEQ ID NO: 253 - protein, 39 aa, Artificial Sequence
  FR3
YADSAKGRFAISRDEAKNMVYLQMNSLKPEDTAVYFCRA

SEQ ID NO: 254 - protein, 39 aa, Artificial Sequence
  FR3
YADFAQGRFTISRDEAKNMVYLQMNSLKPEDTAVYFCRA

SEQ ID NO: 255 - protein, 39 aa, Artificial Sequence
  FR3
YAEFAKGRFTISRDEPKNMVHLQMNSLKPEDTAVYLCRA

SEQ ID NO: 256 - protein, 39 aa, Artificial Sequence
  FR3
YADFAKGRLTISRDEAKNMVYLQMNSLKPEDTAVYFCRA

SEQ ID NO: 257 - protein, 39 aa, Artificial Sequence
  FR3
YADSAKGRFTISRDESKNMVYLQMNSLKPEDTAVYFCRA

SEQ ID NO: 258 - protein, 39 aa, Artificial Sequence
  FR3
YADFAKGRFTISRDGAKNMVYLQMNSLKPEDTAVYFCRA

SEQ ID NO: 259 - protein, 39 aa, Artificial Sequence
  FR3
YADSAKGRFTISRDEARNMVYLQMNSLKPEDTALYFCHA

SEQ ID NO: 260 - protein, 39 aa, Artificial Sequence
  FR3
YADSAKGRFTISRDEAKNMVYLQMNSLKPEDTAAYFCRA

SEQ ID NO: 261 - protein, 39 aa, Artificial Sequence
  FR3
YADSAKGRFTISRDESRNMVYLQMSSLKPEDTAVYFCHA

SEQ ID NO: 262 - protein, 39 aa, Artificial Sequence
  FR3
YADSAKGRFTISRDESRNMVYLQMGSLKPEDTAVYFCHA

SEQ ID NO: 263 - protein, 39 aa, Artificial Sequence
  FR3
YADSAKGRFTISRDEAENMVYLQMNSLKPEDTAVYFCRA

SEQ ID NO: 264 - protein, 39 aa, Artificial Sequence
  FR3
YADSAKGRFTISRDEATNMVYLQMTSLKPEDTAVYFCRA

SEQ ID NO: 265 - protein, 39 aa, Artificial Sequence
  FR3
YAGSAKGRFTISRDEAKNMVYLQLNNLKPEDTAVYFCRA

SEQ ID NO: 266 - protein, 39 aa, Artificial Sequence
  FR3
YADSAKGRFTISRDEAKNMVYLQLNNLKPEDTAVYFCRA

SEQ ID NO: 267 - protein, 39 aa, Artificial Sequence
  FR3
YAEFAKGRFTISRDEPKNMVYLQMNSLKPEDTAVYLCRA

SEQ ID NO: 268 - protein, 39 aa, Artificial Sequence
  FR3
YAHSAKGRFTISRDEAKNMVYLQMTSLKPEDTAVYVCRA

SEQ ID NO: 269 - protein, 39 aa, Artificial Sequence
  FR3
YADFAKGRFTISRDEVKNMVYLQMNSLKPEDTAVYFCRA

SEQ ID NO: 270 - protein, 39 aa, Artificial Sequence
  FR3
YADFAKGRFTISRDEAKNMVYLQMNSLRPEDTAVYFCRA

SEQ ID NO: 271 - protein, 39 aa, Artificial Sequence
  FR3
YSYFAKGRFTISRDEAKNMVYLQMNSLRPEDTAVYFCRA

SEQ ID NO: 272 - protein, 39 aa, Artificial Sequence
  FR3
YADSAKGRFTISRDEAKNVVYLQMNSLKPEDTAVYFCRA

SEQ ID NO: 273 - protein, 39 aa, Artificial Sequence
  FR3
YEDSAKGRFTISRDEAKNMVYLQMTGLKPEDTAVYVCRA

SEQ ID NO: 274 - protein, 39 aa, Artificial Sequence
  FR3
YADSVKGRFTISEDSAKNTVYLQMSSLKPEDTAVYFCNA

SEQ ID NO: 275 - protein, 39 aa, Artificial Sequence
  FR3
YSHFAKGRFTISRDEAKNMVYLQMNGLRPEDTAVYFCRA

SEQ ID NO: 276 - protein, 39 aa, Artificial Sequence
  FR3
YADSAKGRFTISRDEAKNMVYLQMNSLKPEDTAVYLCRA

SEQ ID NO: 277 - protein, 39 aa, Artificial Sequence
  FR3
YAEFAKGRFTISRDEPKNMVYLQMNSLKPVDTAVYLCRA

SEQ ID NO: 278 - protein, 39 aa, Artificial Sequence
  FR3
YSHFAKGRFTISRDEAKNMVYLQMNNLRPEDTAVYFCRA

SEQ ID NO: 279 - protein, 39 aa, Artificial Sequence
  FR3
YADSVKGRFTISEDSAKDTVYLQMNSLKPEDTAVYFCNA

SEQ ID NO: 280 - protein, 39 aa, Artificial Sequence
  FR3
YADSAKGRFTISRDEAKNMVYLQMNSLKPEDAAVYFCRA

SEQ ID NO: 281 - protein, 39 aa, Artificial Sequence
  FR3
YAESAKGRFTISRDESKNMVYLQMNSLKPEDAAVYLCRA

SEQ ID NO: 282 - protein, 39 aa, Artificial Sequence
  FR3
YADSAKGRFTISRDESRNMVYLQMSSLKPENTAVYFCHA

SEQ ID NO: 283 - protein, 39 aa, Artificial Sequence
  FR3
YADSAKGRFTISRDEAKNMVYLQMDSLKPEDTAVYFCRA

SEQ ID NO: 284 - protein, 39 aa, Artificial Sequence
  FR3
YADSAKGRFTISRDEAKNMVYLQMNSLKPGDTAVYFCRA

SEQ ID NO: 285 - protein, 11 aa, Artificial Sequence
  FR4
WGQGTQVTVSS

SEQ ID NO: 286 - protein, 11 aa, Artificial Sequence
  FR4
WGQGTLVTVSS

SEQ ID NO: 287 - protein, 11 aa, Artificial Sequence
  FR4
WGRGTQVTVSS

SEQ ID NO: 288 - protein, 11 aa, Artificial Sequence
  FR4
WGHGTLVTVSS

SEQ ID NO: 289 - protein, 11 aa, Artificial Sequence
  FR4
WGRGTLVTVSS

SEQ ID NO: 290 - protein, 11 aa, Artificial Sequence
  FR4
WDQGTQVTVSS

SEQ ID NO: 291 - protein, 327 aa, Artificial Sequence
  Nanobody sequence
EVQLVESGGGLVQGGGSLSLSCAASGRTFSSYAMAWFRQPPGKEREFVASISWSGENTNYRNSVKGRFTISRDNAKNTVYLQMNSLKPEDTAVYYCAAKIAKTYPDNWYWTKSNNYNYWGQGTLVTVSSGGGGSGGGGSGGGGSGGGGSGGGGSGGGGSGGGGSEVQLVESGGGLVQGGGSLSLSCAASGRTFSSYAMAWFRQPPGKEREFVASISWSGENTNYRNSVKGRFTISRDNAKNTVYLQMNSLKPEDTAVYYCAAKIAKTYPDNWYWTKSNNYNYWGQGTLVTVSSGAADYKDHDGDYKDHDIDYKDDDDKGAAHHHHHH

SEQ ID NO: 292 - protein, 276 aa, Artificial Sequence
  Nanobody sequence
EVQLVESGGGLVQPGGSLRLSCTFSGGTFSSYTMGWFRQAPGKEREFVAEVRWGGVTTYSNSLKDRFSISEDSVKNAVYLQMNSLKPEDTAVYYCAAVRQMYMTVVPDYWGQGTLVTVSSGGGGSEVQLVESGGGLVQPGGSLRLSCAASGSVHKINFLGWYRQAPGKERGLVATITIGDTTDYADYAKGRFTISRDEARNMVYLQMNSLKPEDTAVYFCRAGSRLYPYNYWGQGTLVTVSSGAADYKDHDGDYKDHDIDYKDDDDKGAAHHHHHH

SEQ ID NO: 293 - protein, 289 aa, Artificial Sequence
  Nanobody sequence
EVQLQASGGGSVQAGGSLRLSCAASGYTIGPYCMGWFRQAPGKEREGVAAINMGGGITYYADSVKGRFTISQDNAKNTVYLLMNSLEPEDTAIYYCAADSTIYASYYECGHGLSTGGYGYDSWGQGTQVTVSSGGGGSEVQLVESGGGLVQPGGSLRLSCAASGSVHKINFLGWYRQAPGKERGLVATITIGDTTDYADYAKGRFTISRDEARNMVYLQMNSLKPEDTAVYFCRAGSRLYPYNYWGQGTLVTVSSGAADYKDHDGDYKDHDIDYKDDDDKGAAHHHHHH

SEQ ID NO: 294 - protein, 292 aa, Artificial Sequence
  Nanobody sequence
EVQLVESGGGLVQPGGSLRLSCTFSGGTFSSYTMGWFRQAPGKEREFVAEVRWGGVTTYSNSLKDRFSISEDSVKNAVYLQMNSLKPEDTAVYYCAAVRQMYMTVVPDYWGQGTLVTVSSGGGGSDVQLQASGGGSVQAGGSLRLSCAASGYTIGPYCMGWFRQAPGKEREGVAAINMGGGITYYADSVKGRFTISQDNAKNTVYLLMNSLEPEDTAIYYCAADSTIYASYYECGHGLSTGGYGYDSWGQGTQVTVSSGAADYKDHDGDYKDHDIDYKDDDDKGAAHHHHHH

SEQ ID NO: 295 - protein, 276 aa, Artificial Sequence
  Nanobody sequence
EVQLVESGGGLVQPGGSLRLSCAASGSVHKINFLGWYRQAPGKERGLVATITIGDTTDYADYAKGRFTISRDEARNMVYLQMNSLKPEDTAVYFCRAGSRLYPYNYWGQGTLVTVSSGGGGSEVQLVESGGGLVQPGGSLRLSCTFSGGTFSSYTMGWFRQAPGKEREFVAEVRWGGVTTYSNSLKDRFSISEDSVKNAVYLQMNSLKPEDTAVYYCAAVRQMYMTVVPDYWGQGTLVTVSSGAADYKDHDGDYKDHDIDYKDDDDKGAAHHHHHH

SEQ ID NO: 296 - protein, 280 aa, Artificial Sequence
  Nanobody sequence
EVQLVESGGGLVQPGGSLRLSCTFSGGTFSSYTMGWFRQAPGKEREFVAEVRWGGVTTYSNSLKDRFSISEDSVKNAVYLQMNSLKPEDTAVYYCAAVRQMYMTVVPDYWGQGTLVTVSSGGGGSGGGSEVQLVESGGGLVQPGGSLRLSCAASGSVHKINFLGWYRQAPGKERGLVATITIGDTTDYADYAKGRFTISRDEARNMVYLQMNSLKPEDTAVYFCRAGSRLYPYNYWGQGTLVTVSSGAADYKDHDGDYKDHDIDYKDDDDKGAAHHHHHH

SEQ ID NO: 297 - protein, 293 aa, Artificial Sequence
  Nanobody sequence
EVQLQASGGGSVQAGGSLRLSCAASGYTIGPYCMGWFRQAPGKEREGVAAINMGGGITYYADSVKGRFTISQDNAKNTVYLLMNSLEPEDTAIYYCAADSTIYASYYECGHGLSTGGYGYDSWGQGTQVTVSSGGGGSGGGSEVQLVESGGGLVQPGGSLRLSCAASGSVHKINFLGWYRQAPGKERGLVATITIGDTTDYADYAKGRFTISRDEARNMVYLQMNSLKPEDTAVYFCRAGSRLYPYNYWGQGTLVTVSSGAADYKDHDGDYKDHDIDYKDDDDKGAAHHHHHH

SEQ ID NO: 298 - protein, 296 aa, Artificial Sequence
  Nanobody sequence
EVQLVESGGGLVQPGGSLRLSCTFSGGTFSSYTMGWFRQAPGKEREFVAEVRWGGVTTYSNSLKDRFSISEDSVKNAVYLQMNSLKPEDTAVYYCAAVRQMYMTVVPDYWGQGTLVTVSSGGGGSGGGSDVQLQASGGGSVQAGGSLRLSCAASGYTIGPYCMGWFRQAPGKEREGVAAINMGGGITYYADSVKGRFTISQDNAKNTVYLLMNSLEPEDTAIYYCAADSTIYASYYECGHGLSTGGYGYDSWGQGTQVTVSSGAADYKDHDGDYKDHDIDYKDDDDKGAAHHHHHH

SEQ ID NO: 299 - protein, 280 aa, Artificial Sequence
  Nanobody sequence
EVQLVESGGGLVQPGGSLRLSCAASGSVHKINFLGWYRQAPGKERGLVATITIGDTTDYADYAKGRFTISRDEARNMVYLQMNSLKPEDTAVYFCRAGSRLYPYNYWGQGTLVTVSSGGGGSGGGSEVQLVESGGGLVQPGGSLRLSCTFSGGTFSSYTMGWFRQAPGKEREFVAEVRWGGVTTYSNSLKDRFSISEDSVKNAVYLQMNSLKPEDTAVYYCAAVRQMYMTVVPDYWGQGTLVTVSSGAADYKDHDGDYKDHDIDYKDDDDKGAAHHHHHH

SEQ ID NO: 300 - protein, 306 aa, Artificial Sequence
  Nanobody sequence
EVQLVESGGGLVQPGGSLRLSCTFSGGTFSSYTMGWFRQAPGKEREFVAEVRWGGVTTYSNSLKDRFSISEDSVKNAVYLQMNSLKPEDTAVYYCAAVRQMYMTVVPDYWGQGTLVTVSSGGGGSGGGGSGGGGSGGGGSGGGGSGGGGSGGGGSEVQLVESGGGLVQPGGSLRLSCAASGSVHKINFLGWYRQAPGKERGLVATITIGDTTDYADYAKGRFTISRDEARNMVYLQMNSLKPEDTAVYFCRAGSRLYPYNYWGQGTLVTVSSGAADYKDHDGDYKDHDIDYKDDDDKGAAHHHHHH

SEQ ID NO: 301 - protein, 319 aa, Artificial Sequence
  Nanobody sequence
EVQLQASGGGSVQAGGSLRLSCAASGYTIGPYCMGWFRQAPGKEREGVAAINMGGGITYYADSVKGRFTISQDNAKNTVYLLMNSLEPEDTAIYYCAADSTIYASYYECGHGLSTGGYGYDSWGQGTQVTVSSGGGGSGGGGSGGGGSGGGGSGGGGSGGGGSGGGGSEVQLVESGGGLVQPGGSLRLSCAASGSVHKINFLGWYRQAPGKERGLVATITIGDTTDYADYAKGRFTISRDEARNMVYLQMNSLKPEDTAVYFCRAGSRLYPYNYWGQGTLVTVSSGAADYKDHDGDYKDHDIDYKDDDDKGAAHHHHHH

SEQ ID NO: 302 - protein, 322 aa, Artificial Sequence
  Nanobody sequence
EVQLVESGGGLVQPGGSLRLSCTFSGGTFSSYTMGWFRQAPGKEREFVAEVRWGGVTTYSNSLKDRFSISEDSVKNAVYLQMNSLKPEDTAVYYCAAVRQMYMTVVPDYWGQGTLVTVSSGGGGSGGGGSGGGGSGGGGSGGGGSGGGGSGGGGSDVQLQASGGGSVQAGGSLRLSCAASGYTIGPYCMGWFRQAPGKEREGVAAINMGGGITYYADSVKGRFTISQDNAKNTVYLLMNSLEPEDTAIYYCAADSTIYASYYECGHGLSTGGYGYDSWGQGTQVTVSSGAADYKDHDGDYKDHDIDYKDDDDKGAAHHHHHH

SEQ ID NO: 303 - protein, 306 aa, Artificial Sequence
  Nanobody sequence
EVQLVESGGGLVQPGGSLRLSCAASGSVHKINFLGWYRQAPGKERGLVATITIGDTTDYADYAKGRFTISRDEARNMVYLQMNSLKPEDTAVYFCRAGSRLYPYNYWGQGTLVTVSSGGGGSGGGGSGGGGSGGGGSGGGGSGGGGSGGGGSEVQLVESGGGLVQPGGSLRLSCTFSGGTFSSYTMGWFRQAPGKEREFVAEVRWGGVTTYSNSLKDRFSISEDSVKNAVYLQMNSLKPEDTAVYYCAAVRQMYMTVVPDYWGQGTLVTVSSGAADYKDHDGDYKDHDIDYKDDDDKGAAHHHHHH

SEQ ID NO: 304 - protein, 322 aa, Artificial Sequence
  Nanobody sequence
EVQLQASGGGSVQAGGSLRLSCAASGYTIGPYCMGWFRQAPGKEREGVAAINMGGGITYYADSVKGRFTISQDNAKNTVYLLMNSLEPEDTAIYYCAADSTIYASYYECGHGLSTGGYGYDSWGQGTQVTVSSGGGGSGGGGSGGGGSGGGGSGGGGSGGGGSGGGGSEVQLVESGGGLVQPGGSLRLSCTFSGGTFSSYTMGWFRQAPGKEREFVAEVRWGGVTTYSNSLKDRFSISEDSVKNAVYLQMNSLKPEDTAVYYCAAVRQMYMTVVPDYWGQGTLVTVSSGAADYKDHDGDYKDHDIDYKDDDDKGAAHHHHHH

SEQ ID NO: 305 - protein, 319 aa, Artificial Sequence
  Nanobody sequence
EVQLVESGGGLVQPGGSLRLSCAASGSVHKINFLGWYRQAPGKERGLVATITIGDTTDYADYAKGRFTISRDEARNMVYLQMNSLKPEDTAVYFCRAGSRLYPYNYWGQGTLVTVSSGGGGSGGGGSGGGGSGGGGSGGGGSGGGGSGGGGSDVQLQASGGGSVQAGGSLRLSCAASGYTIGPYCMGWFRQAPGKEREGVAAINMGGGITYYADSVKGRFTISQDNAKNTVYLLMNSLEPEDTAIYYCAADSTIYASYYECGHGLSTGGYGYDSWGQGTQVTVSSGAADYKDHDGDYKDHDIDYKDDDDKGAAHHHHHH

SEQ ID NO: 306 - protein, 306 aa, Artificial Sequence
  Nanobody sequence
EVQLVESGGGLVQPGGSLRLSCAASGDVYKINFLGWHRQAPGKEREKVAHITIGDATDYADSAKGRFTISRDEAKNMVYLQMNSLKPEDTAVYFCRAGSRIYPYDYWGQGTLVTVSSGGGGSGGGGSGGGGSGGGGSGGGGSGGGGSGGGGSEVQLVESGGGLVQPGGSLRLSCTFSGGTFSSYTMGWFRQAPGKEREFVAEVRWGGVTTYSNSLKDRFSISEDSVKNAVYLQMNSLKPEDTAVYYCAAVRQMYMTVVPDYWGQGTLVTVSSGAADYKDHDGDYKDHDIDYKDDDDKGAAHHHHHH

SEQ ID NO: 307 - protein, 306 aa, Artificial Sequence
  Nanobody sequence
EVQLVESGGGLVQPGGSLKLSCAASGAVHKINFLGWYRQTPEKEREMVATITIGDEVDYADSAKGRFTISRDEAKNMVYLQMTSLKPEDTAVYVCRAGSRLYPYNYWGQGTLVTVSSGGGGSGGGGSGGGGSGGGGSGGGGSGGGGSGGGGSEVQLVESGGGLVQPGGSLRLSCTFSGGTFSSYTMGWFRQAPGKEREFVAEVRWGGVTTYSNSLKDRFSISEDSVKNAVYLQMNSLKPEDTAVYYCAAVRQMYMTVVPDYWGQGTLVTVSSGAADYKDHDGDYKDHDIDYKDDDDKGAAHHHHHH

SEQ ID NO: 308 - protein, 306 aa, Artificial Sequence
  Nanobody sequence
EVQLVESGGGLVQPGGSLRLSCITSGETFKINIWGWYRQAPGKQRELVASLTIGGATNYADSVKGRFTISEDSAKNTVYLQMNSLKPEDTAVYFCNAKSRLYPYDYWGQGTLVTVSSGGGGSGGGGSGGGGSGGGGSGGGGSGGGGSGGGGSEVQLVESGGGLVQPGGSLRLSCTFSGGTFSSYTMGWFRQAPGKEREFVAEVRWGGVTTYSNSLKDRFSISEDSVKNAVYLQMNSLKPEDTAVYYCAAVRQMYMTVVPDYWGQGTLVTVSSGAADYKDHDGDYKDHDIDYKDDDDKGAAHHHHHH

SEQ ID NO: 309 - protein, 306 aa, Artificial Sequence
  Nanobody sequence
EVQLVESGGGLVQPGGSLRLSCAASGSVHLLNFLGWYRQAPGKEREMVAHITIADATDYAHFAKGRFTISRDEAKNMVYLQMNSLRPEDTAVYFCRAGSRIYPYDYWGQGTLVTVSSGGGGSGGGGSGGGGSGGGGSGGGGSGGGGSGGGGSEVQLVESGGGLVQPGGSLRLSCTFSGGTFSSYTMGWFRQAPGKEREFVAEVRWGGVTTYSNSLKDRFSISEDSVKNAVYLQMNSLKPEDTAVYYCAAVRQMYMTVVPDYWGQGTLVTVSSGAADYKDHDGDYKDHDIDYKDDDDKGAAHHHHHH

SEQ ID NO: 310 - protein, 306 aa, Artificial Sequence
  Nanobody sequence
EVQLVESGGGLVQPGGSLRLSCITSGETFKINIWGWYRQAPGKQRELVASLTIGGATDYADSVKGRFTISEDSAKNTVYLQMNSLKAEDTAVYFCNAKSRLYPYDYWGQGTLVTVSSGGGGSGGGGSGGGGSGGGGSGGGGSGGGGSGGGGSEVQLVESGGGLVQPGGSLRLSCTFSGGTFSSYTMGWFRQAPGKEREFVAEVRWGGVTTYSNSLKDRFSISEDSVKNAVYLQMNSLKPEDTAVYYCAAVRQMYMTVVPDYWGQGTLVTVSSGAADYKDHDGDYKDHDIDYKDDDDKGAAHHHHHH

SEQ ID NO: 311 - protein, 306 aa, Artificial Sequence
  Nanobody sequence
EVQLVESGGGLVQPGGSLRLSCAASGEVYKINFLGWYRQAPGKEREKVAHITIADAADYADFAKGRFTISRDEAKNMVYLQMNSLRPEDTAVYFCRAGSRIWPYDYWGQGTLVTVSSGGGGSGGGGSGGGGSGGGGSGGGGSGGGGSGGGGSEVQLVESGGGLVQPGGSLRLSCTFSGGTFSSYTMGWFRQAPGKEREFVAEVRWGGVTTYSNSLKDRFSISEDSVKNAVYLQMNSLKPEDTAVYYCAAVRQMYMTVVPDYWGQGTLVTVSSGAADYKDHDGDYKDHDIDYKDDDDKGAAHHHHHH

SEQ ID NO: 312 - protein, 306 aa, Artificial Sequence
  Nanobody sequence
EVQLVESGGGLVQPGGSLRLSCVASGDVHKINFLGWYRQAPGKEREKVAHISIGDQTDYADSAKGRFTISRDESKNMVYLQMNSLKPEDTAVYFCRAFSRIYPYDYWGQGTLVTVSSGGGGSGGGGSGGGGSGGGGSGGGGSGGGGSGGGGSEVQLVESGGGLVQPGGSLRLSCTFSGGTFSSYTMGWFRQAPGKEREFVAEVRWGGVTTYSNSLKDRFSISEDSVKNAVYLQMNSLKPEDTAVYYCAAVRQMYMTVVPDYWGQGTLVTVSSGAADYKDHDGDYKDHDIDYKDDDDKGAAHHHHHH

SEQ ID NO: 313 - protein, 306 aa, Artificial Sequence
  Nanobody sequence
EVQLVESGGGLVQPGGSLRLSCAASGEIGRINFYRWYRQAPGNQREVVATITIADKTDYADSAKGRFTISRDESRNMVYLQMSSLKPEDTAVYFCHAGSRLYPYDYWGQGTLVTVSSGGGGSGGGGSGGGGSGGGGSGGGGSGGGGSGGGGSEVQLVESGGGLVQPGGSLRLSCTFSGGTFSSYTMGWFRQAPGKEREFVAEVRWGGVTTYSNSLKDRFSISEDSVKNAVYLQMNSLKPEDTAVYYCAAVRQMYMTVVPDYWGQGTLVTVSSGAADYKDHDGDYKDHDIDYKDDDDKGAAHHHHHH

SEQ ID NO: 314 - protein, 306 aa, Artificial Sequence
  Nanobody sequence
EVQLVESGGGLVQPGGSLRLSCVASGDVHKINFLGWYRQAPGKEREKVAHITIGDQADYADSAKGRFTISRDEAKNMVYLQMNSLKPEDTAVYFCRAGSRIYPYDYWGQGTLVTVSSGGGGSGGGGSGGGGSGGGGSGGGGSGGGGSGGGGSEVQLVESGGGLVQPGGSLRLSCTFSGGTFSSYTMGWFRQAPGKEREFVAEVRWGGVTTYSNSLKDRFSISEDSVKNAVYLQMNSLKPEDTAVYYCAAVRQMYMTVVPDYWGQGTLVTVSSGAADYKDHDGDYKDHDIDYKDDDDKGAAHHHHHH

SEQ ID NO: 315 - protein, 306 aa, Artificial Sequence
  Nanobody sequence
EVQLVESGGGLVQPGGSLRLSCAASGDVHKINILGWYRQAPAKEREMVAHITIGDATDYADSAKGRFTISRDEAKNMVYLQMNSLKPEDTAVYFCRAYSRIYPYNYWGQGTLVTVSSGGGGSGGGGSGGGGSGGGGSGGGGSGGGGSGGGGSEVQLVESGGGLVQPGGSLRLSCTFSGGTFSSYTMGWFRQAPGKEREFVAEVRWGGVTTYSNSLKDRFSISEDSVKNAVYLQMNSLKPEDTAVYYCAAVRQMYMTVVPDYWGQGTLVTVSSGAADYKDHDGDYKDHDIDYKDDDDKGAAHHHHHH

SEQ ID NO: 316 - protein, 306 aa, Artificial Sequence
  Nanobody sequence
EVQLVESGGGLVQPGGSLRLSCAASGSVHKINFLGWYRQAPGKERELVATITIGDTTDYADSAKGRFTISRDEAKNMVYLQMNSLKPEDTAVYFCRAGSRLYPYNYWGQGTLVTVSSGGGGSGGGGSGGGGSGGGGSGGGGSGGGGSGGGGSEVQLVESGGGLVQPGGSLRLSCTFSGGTFSSYTMGWFRQAPGKEREFVAEVRWGGVTTYSNSLKDRFSISEDSVKNAVYLQMNSLKPEDTAVYYCAAVRQMYMTVVPDYWGQGTLVTVSSGAADYKDHDGDYKDHDIDYKDDDDKGAAHHHHHH

SEQ ID NO: 317 - protein, 306 aa, Artificial Sequence; identical to SEQ ID NO: 303
  Nanobody sequence

SEQ ID NO: 318 - protein, 306 aa, Artificial Sequence
  Nanobody sequence
EVQLVESGGGLVQPGGSLRLSCAASGDVHKINILGWYRQAPAKEREMVAHITIGDATDYADSAKGRFTISRDEAKNMVYLQMNSLKPEDTAVYLCRAYSRIYPYNYWGQGTLVTVSSGGGGSGGGGSGGGGSGGGGSGGGGSGGGGSGGGGSEVQLVESGGGLVQPGGSLRLSCTFSGGTFSSYTMGWFRQAPGKEREFVAEVRWGGVTTYSNSLKDRFSISEDSVKNAVYLQMNSLKPEDTAVYYCAAVRQMYMTVVPDYWGQGTLVTVSSGAADYKDHDGDYKDHDIDYKDDDDKGAAHHHHHH

SEQ ID NO: 319 - protein, 306 aa, Artificial Sequence
  Nanobody sequence
EVQLVESGGGLVQPGGSLRLSCTFSGGTFSSYTMGWFRQAPGKEREFVAEVRWGGVTTYSNSLKDRFSISEDSVKNAVYLQMNSLKPEDTAVYYCAAVRQMYMTVVPDYWGQGTLVTVSSGGGGSGGGGSGGGGSGGGGSGGGGSGGGGSGGGGSEVQLVESGGGLVQPGGSLRLSCVASGDVHKINFLGWYRQAPGKEREKVAHISIGDQTDYADSAKGRFTISRDESKNMVYLQMNSLKPEDTAVYFCRAFSRIYPYDYWGQGTLVTVSSGAADYKDHDGDYKDHDIDYKDDDDKGAAHHHHHH

SEQ ID NO: 320 - protein, 306 aa, Artificial Sequence
  Nanobody sequence
EVQLVESGGGLVQPGGSLRLSCTFSGGTFSSYTMGWFRQAPGKEREFVAEVRWGGVTTYSNSLKDRFSISEDSVKNAVYLQMNSLKPEDTAVYYCAAVRQMYMTVVPDYWGQGTLVTVSSGGGGSGGGGSGGGGSGGGGSGGGGSGGGGSGGGGSEVQLVESGGGLVQPGGSLRLSCAASGEIGRINFYRWYRQAPGNQREVVATITIADKTDYADSAKGRFTISRDESRNMVYLQMSSLKPEDTAVYFCHAGSRLYPYDYWGQGTLVTVSSGAADYKDHDGDYKDHDIDYKDDDDKGAAHHHHHH

SEQ ID NO: 321 - protein, 306 aa, Artificial Sequence
  Nanobody sequence
EVQLVESGGGLVQPGGSLRLSCTFSGGTFSSYTMGWFRQAPGKEREFVAEVRWGGVTTYSNSLKDRFSISEDSVKNAVYLQMNSLKPEDTAVYYCAAVRQMYMTVVPDYWGQGTLVTVSSGGGGSGGGGSGGGGSGGGGSGGGGSGGGGSGGGGSEVQLVESGGGLVQPGGSLRLSCVASGDVHKINFLGWYRQAPGKEREKVAHITIGDQADYADSAKGRFTISRDEAKNMVYLQMNSLKPEDTAVYFCRAGSRIYPYDYWGQGTLVTVSSGAADYKDHDGDYKDHDIDYKDDDDKGAAHHHHHH

SEQ ID NO: 322 - protein, 306 aa, Artificial Sequence
  Nanobody sequence
EVQLVESGGGLVQPGGSLRLSCTFSGGTFSSYTMGWFRQAPGKEREFVAEVRWGGVTTYSNSLKDRFSISEDSVKNAVYLQMNSLKPEDTAVYYCAAVRQMYMTVVPDYWGQGTLVTVSSGGGGSGGGGSGGGGSGGGGSGGGGSGGGGSGGGGSEVQLVESGGGLVQPGGSLRLSCAASGDVHKINILGWYRQAPAKEREMVAHITIGDATDYADSAKGRFTISRDEAKNMVYLQMNSLKPEDTAVYFCRAYSRIYPYNYWGQGTLVTVSSGAADYKDHDGDYKDHDIDYKDDDDKGAAHHHHHH

SEQ ID NO: 323 - protein, 306 aa, Artificial Sequence
  Nanobody sequence
EVQLVESGGGLVQPGGSLRLSCTFSGGTFSSYTMGWFRQAPGKEREFVAEVRWGGVTTYSNSLKDRFSISEDSVKNAVYLQMNSLKPEDTAVYYCAAVRQMYMTVVPDYWGQGTLVTVSSGGGGSGGGGSGGGGSGGGGSGGGGSGGGGSGGGGSEVQLVESGGGLVQPGGSLRLSCAASGSVHKINFLGWYRQAPGKERELVATITIGDTTDYADSAKGRFTISRDEAKNMVYLQMNSLKPEDTAVYFCRAGSRLYPYNYWGQGTLVTVSSGAADYKDHDGDYKDHDIDYKDDDDKGAAHHHHHH

SEQ ID NO: 324 - protein, 306 aa, Artificial Sequence; identical to SEQ ID NO: 300
  Nanobody sequence

SEQ ID NO: 325 - protein, 306 aa, Artificial Sequence
  Nanobody sequence
EVQLVESGGGLVQPGGSLRLSCTFSGGTFSSYTMGWFRQAPGKEREFVAEVRWGGVTTYSNSLKDRFSISEDSVKNAVYLQMNSLKPEDTAVYYCAAVRQMYMTVVPDYWGQGTLVTVSSGGGGSGGGGSGGGGSGGGGSGGGGSGGGGSGGGGSEVQLVESGGGLVQPGGSLRLSCAASGDVYKINFLGWHRQAPGKEREKVAHITIGDATDYADSAKGRFTISRDEAKNMVYLQMNSLKPEDTAVYFCRAGSRIYPYDYWGQGTLVTVSSGAADYKDHDGDYKDHDIDYKDDDDKGAAHHHHHH

SEQ ID NO: 326 - protein, 306 aa, Artificial Sequence
  Nanobody sequence
EVQLVESGGGLVQPGGSLRLSCTFSGGTFSSYTMGWFRQAPGKEREFVAEVRWGGVTTYSNSLKDRFSISEDSVKNAVYLQMNSLKPEDTAVYYCAAVRQMYMTVVPDYWGQGTLVTVSSGGGGSGGGGSGGGGSGGGGSGGGGSGGGGSGGGGSEVQLVESGGGLVQPGGSLRLSCAASGEVYKINFLGWYRQAPGKEREKVAHITIADAADYADFAKGRFTISRDEAKNMVYLQMNSLRPEDTAVYFCRAGSRIWPYDYWGQGTLVTVSSGAADYKDHDGDYKDHDIDYKDDDDKGAAHHHHHH

SEQ ID NO: 327 - protein, 306 aa, Artificial Sequence
  Nanobody sequence
EVQLVESGGGLVQPGGSLRLSCTFSGGTFSSYTMGWFRQAPGKEREFVAEVRWGGVTTYSNSLKDRFSISEDSVKNAVYLQMNSLKPEDTAVYYCAAVRQMYMTVVPDYWGQGTLVTVSSGGGGSGGGGSGGGGSGGGGSGGGGSGGGGSGGGGSEVQLVESGGDLVQPGGSLRLSCAASGDVHKINFLGWYRQAPGKEREMVAHITIADATDYAEFAKGRFTISRDEPKNMVYLQMNSLKPEDTAVYLCRAGSRIYPYNYWGQGTLVTVSSGAADYKDHDGDYKDHDIDYKDDDDKGAAHHHHHH

SEQ ID NO: 328 - protein, 306 aa, Artificial Sequence
  Nanobody sequence
EVQLVESGGGLVQPGGSLRLSCTFSGGTFSSYTMGWFRQAPGKEREFVAEVRWGGVTTYSNSLKDRFSISEDSVKNAVYLQMNSLKPEDTAVYYCAAVRQMYMTVVPDYWGQGTLVTVSSGGGGSGGGGSGGGGSGGGGSGGGGSGGGGSGGGGSEVQLVESGGGLVQPGGSLRLSCITSGETFKINIWGWYRQAPGKQRELVASLTIGGATNYADSVKGRFTISEDSAKNTVYLQMNSLKPEDTAVYFCNAKSRLYPYDYWGQGTLVTVSSGAADYKDHDGDYKDHDIDYKDDDDKGAAHHHHHH

SEQ ID NO: 329 - protein, 306 aa, Artificial Sequence
  Nanobody sequence
EVQLVESGGGLVQPGGSLRLSCTFSGGTFSSYTMGWFRQAPGKEREFVAEVRWGGVTTYSNSLKDRFSISEDSVKNAVYLQMNSLKPEDTAVYYCAAVRQMYMTVVPDYWGQGTLVTVSSGGGGSGGGGSGGGGSGGGGSGGGGSGGGGSGGGGSEVQLVESGGGLVQPGGSLRLSCAASGSVHLLNFLGWYRQAPGKEREMVAHITIADATDYAHFAKGRFTISRDEAKNMVYLQMNSLRPEDTAVYFCRAGSRIYPYDYWGQGTLVTVSSGAADYKDHDGDYKDHDIDYKDDDDKGAAHHHHHH

SEQ ID NO: 330 - protein, 306 aa, Artificial Sequence
  Nanobody sequence
EVQLVESGGGLVQPGGSLRLSCTFSGGTFSSYTMGWFRQAPGKEREFVAEVRWGGVTTYSNSLKDRFSISEDSVKNAVYLQMNSLKPEDTAVYYCAAVRQMYMTVVPDYWGQGTLVTVSSGGGGSGGGGSGGGGSGGGGSGGGGSGGGGSGGGGSEVQLVESGGGLVQPGGSLRLSCITSGETFKINIWGWYRQAPGKQRELVASLTIGGATDYADSVKGRFTISEDSAKNTVYLQMNSLKAEDTAVYFCNAKSRLYPYDYWGQGTLVTVSSGAADYKDHDGDYKDHDIDYKDDDDKGAAHHHHHH

SEQ ID NO: 331 - protein, 306 aa, Artificial Sequence
  Nanobody sequence
EVQLVESGGGLVQPGGSLRLSCAASGDVHKINILGWYRQAPAKEREMVAHITIGDATSYADSAKGRFTISRDEAKNMVYLQLNNLKPEDTAVYFCRAYSRIYPYNYWGQGTLVTVSSGGGGSGGGGSGGGGSGGGGSGGGGSGGGGSGGGGSEVQLVESGGGLVQPGGSLRLSCTFSGGTFSSYTMGWFRQAPGKEREFVAEVRWGGVTTYSNSLKDRFSISEDSVKNAVYLQMNSLKPEDTAVYYCAAVRQMYMTVVPDYWGQGTLVTVSSGAADYKDHDGDYKDHDIDYKDDDDKGAAHHHHHH

SEQ ID NO: 332 - protein, 306 aa, Artificial Sequence; identical to SEQ ID NO: 312
  Nanobody sequence

SEQ ID NO: 333 - protein, 306 aa, Artificial Sequence
  Nanobody sequence
EVQLVESGGGLVQPGGSLRLSCTFSGGTFSSYTMGWFRQAPGKEREFVAEVRWGGVTTYSNSLKDRFSISEDSVKNAVYLQMNSLKPEDTAVYYCAAVRQMYMTVVPDYWGQGTLVTVSSGGGGSGGGGSGGGGSGGGGSGGGGSGGGGSGGGGSEVQLVESGGGLVQPGGSLRLSCAASGDVHKINILGWYRQAPAKEREMVAHITIGDATSYADSAKGRFTISRDEAKNMVYLQLNNLKPEDTAVYFCRAYSRIYPYNYWGQGTLVTVSSGAADYKDHDGDYKDHDIDYKDDDDKGAAHHHHHH

SEQ ID NO: 334 - protein, 306 aa, Artificial Sequence; identical to SEQ ID NO: 319
  Nanobody sequence

SEQ ID NO: 335 - protein, 306 aa, Artificial Sequence
  Nanobody sequence
EVQLVESGGDLVQPGGSLRLSCAASGDVHKINFLGWYRQAPGKEREMVAHITIADATDYAEFAKGRFTISRDEPKNMVYLQMNSLKPEDTAVYLCRAGSRIYPYNYWGQGTLVTVSSGGGGSGGGGSGGGGSGGGGSGGGGSGGGGSGGGGSEVQLVESGGGLVQPGGSLRLSCTFSGGTFSSYTMGWFRQAPGKEREFVAEVRWGGVTTYSNSLKDRFSISEDSVKNAVYLQMNSLKPEDTAVYYCAAVRQMYMTVVPDYWGQGTLVTVSSGAADYKDHDGDYKDHDIDYKDDDDKGAAHHHHHH

SEQ ID NO: 336 - protein, 306 aa, Artificial Sequence
  Nanobody sequence
EVQLVESGGGLVQPGGSLRLSCTFSGGTFSSYTMGWFRQAPGKEREFVAEVRWGGVTTYSNSLKDRFSISEDSVKNAVYLQMNSLKPEDTAVYYCAAVRQMYMTVVPDYWGQGTLVTVSSGGGGSGGGGSGGGGSGGGGSGGGGSGGGGSGGGGSEVQLVESGGGLVQPGGSLRLSCAASGDVHKINILGWYRQAPAKEREMVAHITIGDATDYADSAKGRFTISRDEAKNMVYLQMNSLKPEDTAVYLCRAYSRIYPYNYWGQGTLVTVSSGAADYKDHDGDYKDHDIDYKDDDDKGAAHHHHHH

SEQ ID NO: 337 - protein, 306 aa, Artificial Sequence
  Nanobody sequence
EVQLVESGGGLVQPGGSLRLSCTFSGGTFSSYTMGWFRQAPGKEREFVAEVRWGGVTTYSNSLKDRFSISEDSVKNAVYLQMNSLKPEDTAVYYCAAVRQMYMTVVPDYWGQGTLVTVSSGGGGSGGGGSGGGGSGGGGSGGGGSGGGGSGGGGSEVQLVESGGGLVQPGGSLKLSCAASGAVHKINFLGWYRQTPEKEREMVATITIGDEVDYADSAKGRFTISRDEAKNMVYLQMTSLKPEDTAVYVCRAGSRLYPYNYWGQGTLVTVSSGAADYKDHDGDYKDHDIDYKDDDDKGAAHHHHHH

SEQ ID NO: 338 - protein, 273 aa, Artificial Sequence
  Nanobody sequence
DVQLVESGGGLVQPGGSLRLSCTFSGGTFSSYTMGWFRQAPGKEREFVAEVRWGGVTTYSNSLKDRFSISEDSVKNAVYLQMNSLKPEDTAVYYCAAVRQMYMTVVPDYWGQGTLVTVSSGGGGSGGGGSGGGGSGGGGSGGGGSGGGGSGGGGSEVQLVESGGGLVQPGGSLRLSCAASGDVHKINILGWYRQAPAKEREMVAHITIGDATDYADSAKGRFTISRDEAKNMVYLQMNSLKPEDTAVYFCRAYSRIYPYNYWGQGTLVTVSSA

SEQ ID NO: 339 - protein, 280 aa, Artificial Sequence
  Nanobody sequence
DVQLVESGGGLVQAGDSLRLSCAASGRTFSSYAMGWFRQAPGKEREFVAAISWSDGSTYYADSVKGRFTISRDNAKNTVYLQMNSLKPEDTAVYYCAADLTSTNPGSYIYIWAYDYWGQGTQVTVSSGGGGSGGGGSGGGGSGGGGSGGGGSGGGGSGGGGSEVQLVESGGGLVQPGGSLRLSCAASGDVHKINILGWYRQAPAKEREMVAHITIGDATDYADSAKGRFTISRDEAKNMVYLQMNSLKPEDTAVYFCRAYSRIYPYNYWGQGTLVTVSSA

SEQ ID NO: 340 - protein, 456 aa, Artificial Sequence
  Nanobody sequence
EVQLVESGGGLVQPGGSLRLSCTFSGGTFSSYTMGWFRQAPGKEREFVAEVRWGGVTTYSNSLKDRFSISEDSVKNAVYLQMNSLKPEDTAVYYCAAVRQMYMTVVPDYWGQGTLVTVSSGGGGSGGGGSGGGGSGGGGSGGGGSGGGGSGGGGSEVQLVESGGGLVQPGGSLRLSCVASGDVHKINFLGWYRQAPGKEREKVAHISIGDQTDYADSAKGRFTISRDESKNMVYLQMNSLKPEDTAVYFCRAFSRIYPYDYWGQGTLVTVSSGGGGSGGGGSGGGGSGGGGSGGGGSGGGGSGGGGSEVQLVESGGGLVQPGNSLRLSCAASGFTFSSFGMSWVRQAPGKGLEWVSSISGSGSDTLYADSVKGRFTISRDNAKTTLYLQMNSLRPEDTAVYYCTIGGSLSRSSQGTLVTVSSGAADYKDHDGDYKDHDIDYKDDDDKGAAHHHHHH

SEQ ID NO: 341 - protein, 456 aa, Artificial Sequence
  Nanobody sequence
EVQLVESGGGLVQPGGSLRLSCTFSGGTFSSYTMGWFRQAPGKEREFVAEVRWGGVTTYSNSLKDRFSISEDSVKNAVYLQMNSLKPEDTAVYYCAAVRQMYMTVVPDYWGQGTLVTVSSGGGGSGGGGSGGGGSGGGGSGGGGSGGGGSGGGGSEVQLVESGGGLVQPGGSLRLSCITSGETFKINIWGWYRQAPGKQRELVASLTIGGATNYADSVKGRFTISEDSAKNTVYLQMNSLKPEDTAVYFCNAKSRLYPYDYWGQGTLVTVSSGGGGSGGGGSGGGGSGGGGSGGGGSGGGGSGGGGSEVQLVESGGGLVQPGNSLRLSCAASGFTFSSFGMSWVRQAPGKGLEWVSSISGSGSDTLYADSVKGRFTISRDNAKTTLYLQMNSLRPEDTAVYYCTIGGSLSRSSQGTLVTVSSGAADYKDHDGDYKDHDIDYKDDDDKGAAHHHHHH

SEQ ID NO: 342 - protein, 304 aa, Artificial Sequence
  Nanobody sequence
EVQLVESGGGLVQAGGSLRLSCAASGITFSINTMGWYRQAPGKQRELVALISSIGDTYYADSVKGRFTISRDNAKNTVYLQMNSLKPEDTAVYYCKRFRTAAQGTDYWGQGTLVTVSSGGGGSGGGGSGGGGSGGGGSGGGGSGGGGSGGGGSEVQLVESGGGLVQPGGSLRLSCVASGDVHKINFLGWYRQAPGKEREKVAHISIGDQTDYADSAKGRFTISRDESKNMVYLQMNSLKPEDTAVYFCRAFSRIYPYDYWGQGTLVTVSSGAADYKDHDGDYKDHDIDYKDDDDKGAAHHHHHH

SEQ ID NO: 343 - protein, 304 aa, Artificial Sequence
  Nanobody sequence
EVQLVESGGGLVQPGGSLRLSCVASGDVHKINFLGWYRQAPGKEREKVAHISIGDQTDYADSAKGRFTISRDESKNMVYLQMNSLKPEDTAVYFCRAFSRIYPYDYWGQGTLVTVSSGGGGSGGGGSGGGGSGGGGSGGGGSGGGGSGGGGSEVQLVESGGGLVQAGGSLRLSCAASGITFSINTMGWYRQAPGKQRELVALISSIGDTYYADSVKGRFTISRDNAKNTVYLQMNSLKPEDTAVYYCKRFRTAAQGTDYWGQGTLVTVSSGAADYKDHDGDYKDHDIDYKDDDDKGAAHHHHHH

SEQ ID NO: 344 - protein, 171 aa, Homo sapiens
MEHSTFLSGLVLATLLSQVSPFKIPIEELEDRVFVNCNTSITWVEGTVGTLLSDITRLDLGKRILDPRGIYRCNGTDIYKDKESTVQVHYRMCQSCVELDPATVAGIIVTDVIATLLLALGVFCFAGHETGRLSGAADTQALLRNDQVYQPLRDRDDAQYSHLGGNWARNK

SEQ ID NO: 345 - protein, 182 aa, Homo sapiens
MEQGKGLAVLILAIILLQGTLAQSIKGNHLVKVYDYQEDGSVLLTCDAEAKNITWFKDGKMIGFLTEDKKKWNLGSNAKDPRGMYQCKGSQNKSKPLQVYYRMCQNCIELNAATISGFLFAEIVSIFVLAVGVYFIAGQDGVRQSRASDKQTLLPNDQLYQPLKDREDDQYSHLQGNQLRRN

SEQ ID NO: 346 - protein, 207 aa, Homo sapiens
MQSGTHWRVLGLCLLSVGVWGQDGNEEMGGITQTPYKVSISGTTVILTCPQYPGSEILWQHNDKNIGGDEDDKNIGSDEDHLSLKEFSELEQSGYYVCYPRGSKPEDANFYLYLRARVCENCMEMDVMSVATIVIVDICITGGLLLLVYYWSKNRKAKAKPVTRGAGAGGRQRGQNKERPPPVPNPDYEPIRKGQRDLYSGLNQRRI

SEQ ID NO: 347 - protein, 164 aa, Homo sapiens
MKWKALFTAAILQAQLPITEAQSFGLLDPKLCYLLDGILFIYGVILTALFLRVKFSRSADAPAYQQGQNQLYNELNLGRREEYDVLDKRRGRDPEMGGKPQRRKNPQEGLYNELQKDKMAEAYSEIGMKGERRRGKGHDGLYQGLSTATKDTYDALHMQALPPR

SEQ ID NO: 348 - protein, 142 aa, Homo sapiens
PNIQNPDPAVYQLRDSKSSDKSVCLFTDFDSQTNVSQSKDSDVYITDKTVLDMRSMDFKSNSAVAWSNKSDFACANAFNNSIIPEDTFFPSPESSCDVKLVEKSFETDTNFRILLLKVAGFNLLMTLRLWSSLNFQNLSVIG

SEQ ID NO: 349 - protein, 177 aa, Homo sapiens
EDLNKVFPPEVAVFEPSEAEISHTQKATLVCLATGFFPDHVELSWWVNGKEVHSGVSTDPQPLKEQPALNDSRYCLSSRLRVSATFWQNPRNHFRCQVQFYGLSENDEWTVSAEAWGRADCGFTSVSYQQGVLSATILYEILLGKATLYAVLVSALVLMAMVKRKDFQDRAKPVTQI

SEQ ID NO: 350 - protein, 118 aa, Artificial Sequence
  Nanobody sequence
EVQLVESGGGLVQAGGSLRLSCAASGITFSINTMGWYRQAPGKQRELVALISSIGDTYYADSVKGRFTISRDNAKNTVYLQMNSLKPEDTAVYYCKRFRTAAQGTDYWGQGTLVTVSS

SEQ ID NO: 351 - protein, 119 aa, Artificial Sequence
  Nanobody sequence
EVQLVESGGGLVQPGGSLRLSCAASGSIFGFNDMAWYRQAPGKQRELVALISRVGVTSSADSVKGRFTISRVNAKDTVYLQMNSLKPEDTAVYYCYMDQRLDGSTLAYWGQGTQVTVSS

SEQ ID NO: 352 - protein, 127 aa, Artificial Sequence
  Nanobody sequence
EVQLVESGGGLVQAGGSLRLSCAASGRTFSSYAMGWFRQAPGKEREFVVAINWSSGSTYYADSVKGRFTISRDNAKNTMYLQMNSLKPEDTAVYYCAAGYQINSGNYNFKDYEYDYWGQGTQVTVSS

SEQ ID NO: 353 - protein, 123 aa, Artificial Sequence
  Nanobody sequence
EVQLVESGGGSVQAGGSLRLSCAASGDTYGSYWMGWFRQAPGKEREGVAAINRGGGYTVYADSVKGRFTISRDTAKNTVYLQMNSLRPDDTADYYCAASGVLGGLHEDWFNYWGQGTLVTVSS

SEQ ID NO: 354 - protein, 123 aa, Artificial Sequence
  Nanobody sequence
EVQLVESGGGSVQAGGSLRLSCAASGDTYGSYWMGWFRQAPGQEREAVAAINRGGGYTVYADSVKGRFTISRDNAKNTLYLQMNSLRPDDTADYYCAASGVLGGLHEDWFNYWGQGTLVTVSS

SEQ ID NO: 355 - protein, 124 aa, Artificial Sequence
  Nanobody sequence
EVQLVESGGGSVQTGGSLRLTCAASGRTSRSYGMGWFRQAPGKEREFVSGISWRGDSTGYADSVKGRFTISRDNAKNTVDLQMNSLKPEDTAIYYCAAAAGSAWYGTLYEYDYWGQGTLVTVSS

SEQ ID NO: 356 - protein, 124 aa, Artificial Sequence
  Nanobody sequence
EVQLVESGGGSVQAGGSLRLTCAASGSTSRSYGMGWFRQAPGKEREFVSGISWRGDSTGYADSVKGRFTISRDNAKNTVDLQMNSLKPEDTAIYYCAAAAGSTWYGTLYEYDYWGQGTLVTVSS

SEQ ID NO: 357 - protein, 120 aa, Artificial Sequence
  Nanobody sequence
EVQLVESGGGLVQPGGSLRLSCTFSGGTFSSYTMGWFRQAPGKEREFVAEVRWGGVTTYSNSLKDRFSISEDSVKNAVYLQMNSLKPEDTAVYYCAAVRQMYMTVVPDYWGQGTLVTVSS

SEQ ID NO: 358 - protein, 129 aa, Artificial Sequence
  Nanobody sequence
EVQLVESGGGLVQAGGSLRLSCAASGRTFSSYVMGWFRQATGKEREFVATIAWDSGSTYYADSVKGRFTISRDNAKNTVHLQMNSLKPEDTAVYYCAASYNVYYNNYYYPISRDEYDYWGQGTLVTVSS

SEQ ID NO: 359 - protein, 133 aa, Artificial Sequence
  Nanobody sequence
DVQLQASGGGSVQAGGSLRLSCAASGYTIGPYCMGWFRQAPGKEREGVAAINMGGGITYYADSVKGRFTISQDNAKNTVYLLMNSLEPEDTAIYYCAADSTIYASYYECGHGLSTGGYGYDSWGQGTQVTVSS

SEQ ID NO: 360 - protein, 127 aa, Artificial Sequence
  Nanobody sequence
EVQLVESGGGLVQAGDSLRLSCAASGRTFSSYAMGWFRQAPGKEREFVAAISWSDGSTYYADSVKGRFTISRDNAKNTVYLQMNSLKPEDTAVYYCAADLTSTNPGSYIYIWAYDYWGQGTQVTVSS

SEQ ID NO: 361 - protein, 10 aa, Artificial Sequence
  CDR1
GDTYGSYWMG

SEQ ID NO: 362 - protein, 10 aa, Artificial Sequence
  CDR1
GGTFSSYTMG

SEQ ID NO: 363 - protein, 10 aa, Artificial Sequence
  CDR2
AINRGGGYTV

SEQ ID NO: 364 - protein, 9 aa, Artificial Sequence
  CDR2
EVRWGGVTT

SEQ ID NO: 365 - protein, 14 aa, Artificial Sequence
  CDR3
SGVLGGLHEDWFNY

SEQ ID NO: 366 - protein, 12 aa, Artificial Sequence
  CDR3
VRQMYMTVVPDY

SEQ ID NO: 367 - protein, 25 aa, Artificial Sequence
  FR1
EVQLVESGGGSVQAGGSLRLSCAAS

SEQ ID NO: 368 - protein, 25 aa, Artificial Sequence
  FR1
EVQLVESGGGLVQPGGSLRLSCTFS

SEQ ID NO: 369 - protein, 14 aa, Artificial Sequence
  FR2
WFRQAPGKEREGVA

SEQ ID NO: 370 - protein, 14 aa, Artificial Sequence
  FR2
WFRQAPGQEREAVA

SEQ ID NO: 371 - protein, 14 aa, Artificial Sequence
  FR2
WFRQAPGKEREFVA

SEQ ID NO: 372 - protein, 39 aa, Artificial Sequence
  FR3
YADSVKGRFTISRDTAKNTVYLQMNSLRPDDTADYYCAA

SEQ ID NO: 373 - protein, 39 aa, Artificial Sequence
  FR3
YADSVKGRFTISRDNAKNTLYLQMNSLRPDDTADYYCAA

SEQ ID NO: 374 - protein, 39 aa, Artificial Sequence
  FR3
YSNSLKDRFSISEDSVKNAVYLQMNSLKPEDTAVYYCAA

SEQ ID NO: 375 - protein, 11 aa, Artificial Sequence
  FR4
WGQGTLVTVSS

SEQ ID NO: 376 - protein, 5 aa, Artificial Sequence
  Linker
GGGGS

SEQ ID NO: 377 - protein, 7 aa, Artificial Sequence
  Linker
SGGSGGS

SEQ ID NO: 378 - protein, 9 aa, Artificial Sequence
  Linker
GGGGSGGGS

SEQ ID NO: 379 - protein, 10 aa, Artificial Sequence
  Linker
GGGGSGGGGS

SEQ ID NO: 380 - protein, 15 aa, Artificial Sequence
  Linker
GGGGSGGGGSGGGGS

SEQ ID NO: 381 - protein, 18 aa, Artificial Sequence
  Linker
GGGGSGGGGSGGGGGGGS

SEQ ID NO: 382 - protein, 20 aa, Artificial Sequence
  Linker
GGGGSGGGGSGGGGSGGGGS

SEQ ID NO: 383 - protein, 25 aa, Artificial Sequence
  Linker
GGGGSGGGGSGGGGSGGGGSGGGGS

SEQ ID NO: 384 - protein, 30 aa, Artificial Sequence
  Linker
GGGGSGGGGSGGGGSGGGGSGGGGSGGGGS

SEQ ID NO: 385 - protein, 35 aa, Artificial Sequence
  Linker
GGGGSGGGGSGGGGSGGGGSGGGGSGGGGSGGGGS

SEQ ID NO: 386 - protein, 3 aa, Artificial Sequence
  Linker
AAA

SEQ ID NO: 387 - protein, 423 aa, Artificial Sequence
  Nanobody sequence
DVQLVESGGGLVQPGGSLRLSCTFSGGTFSSYTMGWFRQAPGKEREFVAEVRWGGVTTYSNSLKDRFSISEDSVKNAVYLQMNSLKPEDTAVYYCAAVRQMYMTVVPDYWGQGTLVTVSSGGGGSGGGGSGGGGSGGGGSGGGGSGGGGSGGGGSEVQLVESGGGLVQPGGSLRLSCAASGDVHKINILGWYRQAPAKEREMVAHITIGDATDYADSAKGRFTISRDEAKNMVYLQMNSLKPEDTAVYFCRAYSRIYPYNYWGQGTLVTVSSGGGGSGGGGSGGGGSGGGGSGGGGSGGGGSGGGGSEVQLVESGGGLVQPGNSLRLSCAASGFTFSSFGMSWVRQAPGKGLEWVSSISGSGSDTLYADSVKGRFTISRDNAKTTLYLQMNSLRPEDTAVYYCTIGGSLSRSSQGTLVTVSSA

SEQ ID NO: 388 - protein, 273 aa, Artificial Sequence
  Nanobody sequence
DVQLVESGGGLVQPGGSLRLSCTFSGGTFSSYTMGWFRQAPGKEREFVAEVRWGGVTTYSNSLKDRFSISEDSVKNAVYLQMNSLKPEDTAVYYCAAVRQMYMTVVPDYWGQGTLVTVSSGGGGSGGGGSGGGGSGGGGSGGGGSGGGGSGGGGSEVQLVESGGGLVQPGGSLRLSCVASGDVHKINFLGWYRQAPGKEREKVAHISIGDQTDYADSAKGRFTISRDESKNMVYLQMNSLKPEDTAVYFCRAFSRIYPYDYWGQGTLVTVSSA

SEQ ID NO: 389 - protein, 430 aa, Artificial Sequence
  Nanobody sequence
DVQLVESGGGLVQAGDSLRLSCAASGRTFSSYAMGWFRQAPGKEREFVAAISWSDGSTYYADSVKGRFTISRDNAKNTVYLQMNSLKPEDTAVYYCAADLTSTNPGSYIYIWAYDYWGQGTQVTVSSGGGGSGGGGSGGGGSGGGGSGGGGSGGGGSGGGGSEVQLVESGGGLVQPGGSLRLSCAASGDVHKINILGWYRQAPAKEREMVAHITIGDATDYADSAKGRFTISRDEAKNMVYLQMNSLKPEDTAVYFCRAYSRIYPYNYWGQGTLVTVSSGGGGSGGGGSGGGGSGGGGSGGGGSGGGGSGGGGSEVQLVESGGGLVQPGNSLRLSCAASGFTFSSFGMSWVRQAPGKGLEWVSSISGSGSDTLYADSVKGRFTISRDNAKTTLYLQMNSLRPEDTAVYYCTIGGSLSRSSQGTLVTVSSA

SEQ ID NO: 390 - protein, 473 aa, Artificial Sequence
  Nanobody sequence
EVQLVESGGGLVQAGGSLRLSCAASGRTFSSYVMGWFRQATGKEREFVATIAWDSGSTYYADSVKGRFTISRDNAKNTVHLQMNSLKPEDTAVYYCAASYNVYYNNYYYPISRDEYDYWGQGTLVTVSSGGGGSGGGGSGGGGSGGGGSGGGGSGGGGSGGGGSEVQLVESGGGSVQAGGSLRLSCAASGDTYGSYWMGWFRQAPGKEREGVAAINRGGGYTVYADSVKGRFTISRDTAKNTVYLQMNSLRPDDTADYYCAASGVLGGLHEDWFNYWGQGTLVTVSSGGGGSGGGGSGGGGSGGGGSGGGGSGGGGSGGGGSEVQLVESGGGLVQPGGSLRLSCVASGDVHKINFLGWYRQAPGKEREKVAHISIGDQTDYADSAKGRFTISRDESKNMVYLQMNSLKPEDTAVYFCRAFSRIYPYDYWGQGTLVTVSSGAADYKDHDGDYKDHDIDYKDDDDKGAAHHHHHH

SEQ ID NO: 391 - protein, 477 aa, Artificial Sequence
  Nanobody sequence
EVQLVESGGGSVQAGGSLRLSCAASGYTIGPYCMGWFRQAPGKEREGVAAINMGGGITYYADSVKGRFTISQDNAKNTVYLLMNSLEPEDTAIYYCAADSTIYASYYECGHGLSTGGYGYDSWGQGTLVTVSSGGGGSGGGGSGGGGSGGGGSGGGGSGGGGSGGGGSEVQLVESGGGSVQAGGSLRLSCAASGDTYGSYWMGWFRQAPGKEREGVAAINRGGGYTVYADSVKGRFTISRDTAKNTVYLQMNSLRPDDTADYYCAASGVLGGLHEDWFNYWGQGTLVTVSSGGGGSGGGGSGGGGSGGGGSGGGGSGGGGSGGGGSEVQLVESGGGLVQPGGSLRLSCVASGDVHKINFLGWYRQAPGKEREKVAHISIGDQTDYADSAKGRFTISRDESKNMVYLQMNSLKPEDTAVYFCRAFSRIYPYDYWGQGTLVTVSSGAADYKDHDGDYKDHDIDYKDDDDKGAAHHHHHH

SEQ ID NO: 392 - protein, 483 aa, Artificial Sequence
  Nanobody sequence
EVQLVESGGGLVQAGGSLRLSCAASGRTFSSYVMGWFRQATGKEREFVATIAWDSGSTYYADSVKGRFTISRDNAKNTVHLQMNSLKPEDTAVYYCAASYNVYYNNYYYPISRDEYDYWGQGTLVTVSSGGGGSGGGGSGGGGSGGGGSGGGGSGGGGSGGGGSEVQLVESGGGSVQAGGSLRLSCAASGYTIGPYCMGWFRQAPGKEREGVAAINMGGGITYYADSVKGRFTISQDNAKNTVYLLMNSLEPEDTAIYYCAADSTIYASYYECGHGLSTGGYGYDSWGQGTLVTVSSGGGGSGGGGSGGGGSGGGGSGGGGSGGGGSGGGGSEVQLVESGGGLVQPGGSLRLSCVASGDVHKINFLGWYRQAPGKEREKVAHISIGDQTDYADSAKGRFTISRDESKNMVYLQMNSLKPEDTAVYFCRAFSRIYPYDYWGQGTLVTVSSGAADYKDHDGDYKDHDIDYKDDDDKGAAHHHHHH

SEQ ID NO: 393 - protein, 107 aa, Homo sapiens
IQVEQSPPDLILQEGANSTLRCNFSDSVNNLQWFHQNPWGQLINLFYIPSGTKQNGRLSATTVATERYSLLYISSSQTTDSGVYFCAALIQGAQKLVFGQGTRLTIN

SEQ ID NO: 394 - protein, 108 aa, Homo sapiens
QLLEQSPQFLSIQEGENLTVYCNSSSVFSSLQWYRQEPGEGPVLLVTVVTGGEVKKLKRLTFQFGDARKDSSLHITAAQPGDTGLYLCAGAGSQGNLIFGKGTKLSVK

SEQ ID NO: 395 - protein, 110 aa, Homo sapiens
GDAKTTQPNSMESNEEEPVHLPCNHSTISGTDYIHWYRQLPSQGPEYVIHGLTSNVNNRMASLAIAEDRKSSTLILHRATLRDAAVYYCTVYGGATNKLIFGTGTLLAVQ

SEQ ID NO: 396 - protein, 96 aa, Macaca fascicularis
PYIQNPDPAVYQLRGSKSNDTSVCLFTDFDSVMNVSQSKDSDVHITDKTVLDMRSMDFKSNGAVAWSNKSDFACTSAFKDSVIPADTFFPSPESSC

SEQ ID NO: 397 - protein, 131 aa, Macaca mulatta
EDLKKVFPPKVAVFEPSEAEISHTQKATLVCLATGFYPDHVELSWWVNGKEVHSGVSTDPQPLKEQPALEDSRYSLSSRLRVSATFWHNPRNHFRCQVQFYGLSEDDEWTEDRDKPITQKISAEAWGRADC

SEQ ID NO: 398 - protein, 107 aa, Macaca mulatta
QQIMQIPQYQHVQEGEDFTTYCNSSTTLSNIQWYKQRPGGHPVFLIMLVKSGEVKKQKRLIFQFGEAKKNSSLHITATQTTDVGTYFCATTGVNNLFFGTGTRLTVL

SEQ ID NO: 399 - protein, 118 aa, Macaca mulatta
AGPVNAGVTQTPKFQVLKTGQSMTLQCAQDMNHDYMYWYRQDPGMGLRLIHYSVGEGSTEKGEVPDGYNVTRSNTEDFPLRLESAAPSQTSVYFCASSYWTGRSYEQYFGPGTRLTVI

SEQ ID NO: 400 - protein, 115 aa, Artificial Sequence [sequence omitted]

SEQ ID NO: 401 - protein, 115 aa, Artificial Sequence [sequence omitted]

SEQ ID NO: 402 - protein, 116 aa, Artificial Sequence
  Nanobody sequence
EVQLVESGGGVVQPGNSLRLSCAASGFTFSSFGMSWVRQAPGKGLEWVSSISGSGSDTLYADSVKGRFTISRDNAKTTLYLQMNSLRPEDTATYYCTIGGSLSRSSQGTLVTVSSA

SEQ ID NO: 403 - protein, 116 aa, Artificial Sequence
  Nanobody sequence
EVQLVESGGGVVQPGGSLRLSCAASGFTFRSFGMSWVRQAPGKGPEWVSSISGSGSDTLYADSVKGRFTISRDNSKNTLYLQMNSLRPEDTATYYCTIGGSLSRSSQGTLVTVSSA

SEQ ID NO: 404 - protein, 115 aa, Artificial Sequence [sequence omitted]

SEQ ID NO: 405 - protein, 116 aa, Artificial Sequence
  Nanobody sequence
EVQLVESGGGLVQPGNSLRLSCAASGFTFSSFGMSWVRQAPGKGLEWVSSISGSGSDTLYADSVKGRFTISRDNAKTTLYLQMNSLRPEDTAVYYCTIGGSLSRSSQGTLVKVSSA

SEQ ID NO: 406 - protein, 115 aa, Artificial Sequence
  Nanobody sequence
EVQLVESGGGVVQPGNSLRLSCAASGFTFSSFGMSWVRQAPGKGLEWVSSISGSGSDTLYADSVKGRFTISRDNAKTTLYLQMNSLRPEDTALYYCTIGGSLSRSSQGTLVTVSS

SEQ ID NO: 407 - protein, 116 aa, Artificial Sequence
  Nanobody sequence
EVQLVESGGGVVQPGNSLRLSCAASGFTFSSFGMSWVRQAPGKGLEWVSSISGSGSDTLYADSVKGRFTISRDNAKTTLYLQMNSLRPEDTALYYCTIGGSLSRSSQGTLVTVSSA

SEQ ID NO: 408 - protein, 117 aa, Artificial Sequence
  Nanobody sequence
EVQLVESGGGVVQPGNSLRLSCAASGFTFSSFGMSWVRQAPGKGLEWVSSISGSGSDTLYADSVKGRFTISRDNAKTTLYLQMNSLRPEDTALYYCTIGGSLSRSSQGTLVTVSSAA

SEQ ID NO: 409 - protein, 118 aa, Artificial Sequence
  Nanobody sequence
EVQLVESGGGVVQPGNSLRLSCAASGFTFSSFGMSWVRQAPGKGLEWVSSISGSGSDTLYADSVKGRFTISRDNAKTTLYLQMNSLRPEDTALYYCTIGGSLSRSSQGTLVTVSSAAA

SEQ ID NO: 410 - protein, 116 aa, Artificial Sequence
  Nanobody sequence
EVQLVESGGGVVQPGNSLRLSCAASGFTFSSFGMSWVRQAPGKGLEWVSSISGSGSDTLYADSVKGRFTISRDNAKTTLYLQMNSLRPEDTALYYCTIGGSLSRSSQGTLVTVSSG

SEQ ID NO: 411 - protein, 117 aa, Artificial Sequence
  Nanobody sequence
EVQLVESGGGVVQPGNSLRLSCAASGFTFSSFGMSWVRQAPGKGLEWVSSISGSGSDTLYADSVKGRFTISRDNAKTTLYLQMNSLRPEDTALYYCTIGGSLSRSSQGTLVTVSSGG

SEQ ID NO: 412 - protein, 118 aa, Artificial Sequence
  Nanobody sequence
EVQLVESGGGVVQPGNSLRLSCAASGFTFSSFGMSWVRQAPGKGLEWVSSISGSGSDTLYADSVKGRFTISRDNAKTTLYLQMNSLRPEDTALYYCTIGGSLSRSSQGTLVTVSSGGG

SEQ ID NO: 413 - protein, 293 aa, Artificial Sequence
  Nanobody sequence
EVQLVESGGGLVQGGGSLSLSCAASGRTFSSYAMAWFRQPPGKEREFVASISWSGENTNYRNSVKGRFTISRDNAKNTVYLQMNSLKPEDTAVYYCAAKIAKTYPDNWYWTKSNNYNYWGQGTLVTVSSGGGGSGGGGSGGGGSGGGGSGGGGSGGGGSGGGGSEVQLVESGGGLVQGGGSLSLSCAASGRTFSSYAMAWFRQPPGKEREFVASISWSGENTNYRNSVKGRFTISRDNAKNTVYLQMNSLKPEDTAVYYCAAKIAKTYPDNWYWTKSNNYNYWGQGTLVTVSS

SEQ ID NO: 414 - protein, 242 aa, Artificial Sequence
  Nanobody sequence
EVQLVESGGGLVQPGGSLRLSCTFSGGTFSSYTMGWFRQAPGKEREFVAEVRWGGVTTYSNSLKDRFSISEDSVKNAVYLQMNSLKPEDTAVYYCAAVRQMYMTVVPDYWGQGTLVTVSSGGGGSEVQLVESGGGLVQPGGSLRLSCAASGSVHKINFLGWYRQAPGKERGLVATITIGDTTDYADYAKGRFTISRDEARNMVYLQMNSLKPEDTAVYFCRAGSRLYPYNYWGQGTLVTVSS

SEQ ID NO: 415 - protein, 255 aa, Artificial Sequence
  Nanobody sequence
EVQLQASGGGSVQAGGSLRLSCAASGYTIGPYCMGWFRQAPGKEREGVAAINMGGGITYYADSVKGRFTISQDNAKNTVYLLMNSLEPEDTAIYYCAADSTIYASYYECGHGLSTGGYGYDSWGQGTQVTVSSGGGGSEVQLVESGGGLVQPGGSLRLSCAASGSVHKINFLGWYRQAPGKERGLVATITIGDTTDYADYAKGRFTISRDEARNMVYLQMNSLKPEDTAVYFCRAGSRLYPYNYWGQGTLVTVSS

SEQ ID NO: 416 - protein, 258 aa, Artificial Sequence
  Nanobody sequence
EVQLVESGGGLVQPGGSLRLSCTFSGGTFSSYTMGWFRQAPGKEREFVAEVRWGGVTTYSNSLKDRFSISEDSVKNAVYLQMNSLKPEDTAVYYCAAVRQMYMTVVPDYWGQGTLVTVSSGGGGSDVQLQASGGGSVQAGGSLRLSCAASGYTIGPYCMGWFRQAPGKEREGVAAINMGGGITYYADSVKGRFTISQDNAKNTVYLLMNSLEPEDTAIYYCAADSTIYASYYECGHGLSTGGYGYDSWGQGTQVTVSS

SEQ ID NO: 417 - protein, 242 aa, Artificial Sequence
  Nanobody sequence
EVQLVESGGGLVQPGGSLRLSCAASGSVHKINFLGWYRQAPGKERGLVATITIGDTTDYADYAKGRFTISRDEARNMVYLQMNSLKPEDTAVYFCRAGSRLYPYNYWGQGTLVTVSSGGGGSEVQLVESGGGLVQPGGSLRLSCTFSGGTFSSYTMGWFRQAPGKEREFVAEVRWGGVTTYSNSLKDRFSISEDSVKNAVYLQMNSLKPEDTAVYYCAAVRQMYMTVVPDYWGQGTLVTVSS

SEQ ID NO: 418 - protein, 246 aa, Artificial Sequence
  Nanobody sequence
EVQLVESGGGLVQPGGSLRLSCTFSGGTFSSYTMGWFRQAPGKEREFVAEVRWGGVTTYSNSLKDRFSISEDSVKNAVYLQMNSLKPEDTAVYYCAAVRQMYMTVVPDYWGQGTLVTVSSGGGGSGGGSEVQLVESGGGLVQPGGSLRLSCAASGSVHKINFLGWYRQAPGKERGLVATITIGDTTDYADYAKGRFTISRDEARNMVYLQMNSLKPEDTAVYFCRAGSRLYPYNYWGQGTLVTVSS

SEQ ID NO: 419 - protein, 259 aa, Artificial Sequence
  Nanobody sequence
EVQLQASGGGSVQAGGSLRLSCAASGYTIGPYCMGWFRQAPGKEREGVAAINMGGGITYYADSVKGRFTISQDNAKNTVYLLMNSLEPEDTAIYYCAADSTIYASYYECGHGLSTGGYGYDSWGQGTQVTVSSGGGGSGGGSEVQLVESGGGLVQPGGSLRLSCAASGSVHKINFLGWYRQAPGKERGLVATITIGDTTDYADYAKGRFTISRDEARNMVYLQMNSLKPEDTAVYFCRAGSRLYPYNYWGQGTLVTVSS

SEQ ID NO: 420 - protein, 262 aa, Artificial Sequence
  Nanobody sequence
EVQLVESGGGLVQPGGSLRLSCTFSGGTFSSYTMGWFRQAPGKEREFVAEVRWGGVTTYSNSLKDRFSISEDSVKNAVYLQMNSLKPEDTAVYYCAAVRQMYMTVVPDYWGQGTLVTVSSGGGGSGGGSDVQLQASGGGSVQAGGSLRLSCAASGYTIGPYCMGWFRQAPGKEREGVAAINMGGGITYYADSVKGRFTISQDNAKNTVYLLMNSLEPEDTAIYYCAADSTIYASYYECGHGLSTGGYGYDSWGQGTQVTVSS

SEQ ID NO: 421 - protein, 246 aa, Artificial Sequence
  Nanobody sequence
EVQLVESGGGLVQPGGSLRLSCAASGSVHKINFLGWYRQAPGKERGLVATITIGDTTDYADYAKGRFTISRDEARNMVYLQMNSLKPEDTAVYFCRAGSRLYPYNYWGQGTLVTVSSGGGGSGGGSEVQLVESGGGLVQPGGSLRLSCTFSGGTFSSYTMGWFRQAPGKEREFVAEVRWGGVTTYSNSLKDRFSISEDSVKNAVYLQMNSLKPEDTAVYYCAAVRQMYMTVVPDYWGQGTLVTVSS

SEQ ID NO: 422 - protein, 272 aa, Artificial Sequence
  Nanobody sequence
EVQLVESGGGLVQPGGSLRLSCTFSGGTFSSYTMGWFRQAPGKEREFVAEVRWGGVTTYSNSLKDRFSISEDSVKNAVYLQMNSLKPEDTAVYYCAAVRQMYMTVVPDYWGQGTLVTVSSGGGGSGGGGSGGGGSGGGGSGGGGSGGGGSGGGGSEVQLVESGGGLVQPGGSLRLSCAASGSVHKINFLGWYRQAPGKERGLVATITIGDTTDYADYAKGRFTISRDEARNMVYLQMNSLKPEDTAVYFCRAGSRLYPYNYWGQGTLVTVSS

SEQ ID NO: 423 - protein, 285 aa, Artificial Sequence
  Nanobody sequence
EVQLQASGGGSVQAGGSLRLSCAASGYTIGPYCMGWFRQAPGKEREGVAAINMGGGITYYADSVKGRFTISQDNAKNTVYLLMNSLEPEDTAIYYCAADSTIYASYYECGHGLSTGGYGYDSWGQGTQVTVSSGGGGSGGGGSGGGGSGGGGSGGGGSGGGGSGGGGSEVQLVESGGGLVQPGGSLRLSCAASGSVHKINFLGWYRQAPGKERGLVATITIGDTTDYADYAKGRFTISRDEARNMVYLQMNSLKPEDTAVYFCRAGSRLYPYNYWGQGTLVTVSS

SEQ ID NO: 424 - protein, 288 aa, Artificial Sequence
  Nanobody sequence
EVQLVESGGGLVQPGGSLRLSCTFSGGTFSSYTMGWFRQAPGKEREFVAEVRWGGVTTYSNSLKDRFSISEDSVKNAVYLQMNSLKPEDTAVYYCAAVRQMYMTVVPDYWGQGTLVTVSSGGGGSGGGGSGGGGSGGGGSGGGGSGGGGSGGGGSDVQLQASGGGSVQAGGSLRLSCAASGYTIGPYCMGWFRQAPGKEREGVAAINMGGGITYYADSVKGRFTISQDNAKNTVYLLMNSLEPEDTAIYYCAADSTIYASYYECGHGLSTGGYGYDSWGQGTQVTVSS

SEQ ID NO: 425 - protein, 272 aa, Artificial Sequence
  Nanobody sequence
EVQLVESGGGLVQPGGSLRLSCAASGSVHKINFLGWYRQAPGKERGLVATITIGDTTDYADYAKGRFTISRDEARNMVYLQMNSLKPEDTAVYFCRAGSRLYPYNYWGQGTLVTVSSGGGGSGGGGSGGGGSGGGGSGGGGSGGGGSGGGGSEVQLVESGGGLVQPGGSLRLSCTFSGGTFSSYTMGWFRQAPGKEREFVAEVRWGGVTTYSNSLKDRFSISEDSVKNAVYLQMNSLKPEDTAVYYCAAVRQMYMTVVPDYWGQGTLVTVSS

SEQ ID NO: 426 - protein, 288 aa, Artificial Sequence
  Nanobody sequence
EVQLQASGGGSVQAGGSLRLSCAASGYTIGPYCMGWFRQAPGKEREGVAAINMGGGITYYADSVKGRFTISQDNAKNTVYLLMNSLEPEDTAIYYCAADSTIYASYYECGHGLSTGGYGYDSWGQGTQVTVSSGGGGSGGGGSGGGGSGGGGSGGGGSGGGGSGGGGSEVQLVESGGGLVQPGGSLRLSCTFSGGTFSSYTMGWFRQAPGKEREFVAEVRWGGVTTYSNSLKDRFSISEDSVKNAVYLQMNSLKPEDTAVYYCAAVRQMYMTVVPDYWGQGTLVTVSS

SEQ ID NO: 427 - protein, 285 aa, Artificial Sequence
  Nanobody sequence
EVQLVESGGGLVQPGGSLRLSCAASGSVHKINFLGWYRQAPGKERGLVATITIGDTTDYADYAKGRFTISRDEARNMVYLQMNSLKPEDTAVYFCRAGSRLYPYNYWGQGTLVTVSSGGGGSGGGGSGGGGSGGGGSGGGGSGGGGSGGGGSDVQLQASGGGSVQAGGSLRLSCAASGYTIGPYCMGWFRQAPGKEREGVAAINMGGGITYYADSVKGRFTISQDNAKNTVYLLMNSLEPEDTAIYYCAADSTIYASYYECGHGLSTGGYGYDSWGQGTQVTVSS

SEQ ID NO: 428 - protein, 272 aa, Artificial Sequence
  Nanobody sequence
EVQLVESGGGLVQPGGSLRLSCAASGDVYKINFLGWHRQAPGKEREKVAHITIGDATDYADSAKGRFTISRDEAKNMVYLQMNSLKPEDTAVYFCRAGSRIYPYDYWGQGTLVTVSSGGGGSGGGGSGGGGSGGGGSGGGGSGGGGSGGGGSEVQLVESGGGLVQPGGSLRLSCTFSGGTFSSYTMGWFRQAPGKEREFVAEVRWGGVTTYSNSLKDRFSISEDSVKNAVYLQMNSLKPEDTAVYYCAAVRQMYMTVVPDYWGQGTLVTVSS

SEQ ID NO: 429 - protein, 272 aa, Artificial Sequence
  Nanobody sequence
EVQLVESGGGLVQPGGSLKLSCAASGAVHKINFLGWYRQTPEKEREMVATITIGDEVDYADSAKGRFTISRDEAKNMVYLQMTSLKPEDTAVYVCRAGSRLYPYNYWGQGTLVTVSSGGGGSGGGGSGGGGSGGGGSGGGGSGGGGSGGGGSEVQLVESGGGLVQPGGSLRLSCTFSGGTFSSYTMGWFRQAPGKEREFVAEVRWGGVTTYSNSLKDRFSISEDSVKNAVYLQMNSLKPEDTAVYYCAAVRQMYMTVVPDYWGQGTLVTVSS

SEQ ID NO: 430 - protein, 272 aa, Artificial Sequence
  Nanobody sequence
EVQLVESGGGLVQPGGSLRLSCITSGETFKINIWGWYRQAPGKQRELVASLTIGGATNYADSVKGRFTISEDSAKNTVYLQMNSLKPEDTAVYFCNAKSRLYPYDYWGQGTLVTVSSGGGGSGGGGSGGGGSGGGGSGGGGSGGGGSGGGGSEVQLVESGGGLVQPGGSLRLSCTFSGGTFSSYTMGWFRQAPGKEREFVAEVRWGGVTTYSNSLKDRFSISEDSVKNAVYLQMNSLKPEDTAVYYCAAVRQMYMTVVPDYWGQGTLVTVSS

SEQ ID NO: 431 - protein, 272 aa, Artificial Sequence
  Nanobody sequence
EVQLVESGGGLVQPGGSLRLSCAASGSVHLLNFLGWYRQAPGKEREMVAHITIADATDYAHFAKGRFTISRDEAKNMVYLQMNSLRPEDTAVYFCRAGSRIYPYDYWGQGTLVTVSSGGGGSGGGGSGGGGSGGGGSGGGGSGGGGSGGGGSEVQLVESGGGLVQPGGSLRLSCTFSGGTFSSYTMGWFRQAPGKEREFVAEVRWGGVTTYSNSLKDRFSISEDSVKNAVYLQMNSLKPEDTAVYYCAAVRQMYMTVVPDYWGQGTLVTVSS

SEQ ID NO: 432 - protein, 272 aa, Artificial Sequence
  Nanobody sequence
EVQLVESGGGLVQPGGSLRLSCITSGETFKINIWGWYRQAPGKQRELVASLTIGGATDYADSVKGRFTISEDSAKNTVYLQMNSLKAEDTAVYFCNAKSRLYPYDYWGQGTLVTVSSGGGGSGGGGSGGGGSGGGGSGGGGSGGGGSGGGGSEVQLVESGGGLVQPGGSLRLSCTFSGGTFSSYTMGWFRQAPGKEREFVAEVRWGGVTTYSNSLKDRFSISEDSVKNAVYLQMNSLKPEDTAVYYCAAVRQMYMTVVPDYWGQGTLVTVSS

SEQ ID NO: 433 - protein, 272 aa, Artificial Sequence
  Nanobody sequence
EVQLVESGGGLVQPGGSLRLSCAASGEVYKINFLGWYRQAPGKEREKVAHITIADAADYADFAKGRFTISRDEAKNMVYLQMNSLRPEDTAVYFCRAGSRIWPYDYWGQGTLVTVSSGGGGSGGGGSGGGGSGGGGSGGGGSGGGGSGGGGSEVQLVESGGGLVQPGGSLRLSCTFSGGTFSSYTMGWFRQAPGKEREFVAEVRWGGVTTYSNSLKDRFSISEDSVKNAVYLQMNSLKPEDTAVYYCAAVRQMYMTVVPDYWGQGTLVTVSS

SEQ ID NO: 434 - protein, 272 aa, Artificial Sequence
  Nanobody sequence
EVQLVESGGGLVQPGGSLRLSCVASGDVHKINFLGWYRQAPGKEREKVAHISIGDQTDYADSAKGRFTISRDESKNMVYLQMNSLKPEDTAVYFCRAFSRIYPYDYWGQGTLVTVSSGGGGSGGGGSGGGGSGGGGSGGGGSGGGGSGGGGSEVQLVESGGGLVQPGGSLRLSCTFSGGTFSSYTMGWFRQAPGKEREFVAEVRWGGVTTYSNSLKDRFSISEDSVKNAVYLQMNSLKPEDTAVYYCAAVRQMYMTVVPDYWGQGTLVTVSS

SEQ ID NO: 435 - protein, 272 aa, Artificial Sequence
  Nanobody sequence
EVQLVESGGGLVQPGGSLRLSCAASGEIGRINFYRWYRQAPGNQREVVATITIADKTDYADSAKGRFTISRDESRNMVYLQMSSLKPEDTAVYFCHAGSRLYPYDYWGQGTLVTVSSGGGGSGGGGSGGGGSGGGGSGGGGSGGGGSGGGGSEVQLVESGGGLVQPGGSLRLSCTFSGGTFSSYTMGWFRQAPGKEREFVAEVRWGGVTTYSNSLKDRFSISEDSVKNAVYLQMNSLKPEDTAVYYCAAVRQMYMTVVPDYWGQGTLVTVSS

SEQ ID NO: 436 - protein, 272 aa, Artificial Sequence
  Nanobody sequence
EVQLVESGGGLVQPGGSLRLSCVASGDVHKINFLGWYRQAPGKEREKVAHITIGDQADYADSAKGRFTISRDEAKNMVYLQMNSLKPEDTAVYFCRAGSRIYPYDYWGQGTLVTVSSGGGGSGGGGSGGGGSGGGGSGGGGSGGGGSGGGGSEVQLVESGGGLVQPGGSLRLSCTFSGGTFSSYTMGWFRQAPGKEREFVAEVRWGGVTTYSNSLKDRFSISEDSVKNAVYLQMNSLKPEDTAVYYCAAVRQMYMTVVPDYWGQGTLVTVSS

SEQ ID NO: 437 - protein, 272 aa, Artificial Sequence
  Nanobody sequence
EVQLVESGGGLVQPGGSLRLSCAASGDVHKINILGWYRQAPAKEREMVAHITIGDATDYADSAKGRFTISRDEAKNMVYLQMNSLKPEDTAVYFCRAYSRIYPYNYWGQGTLVTVSSGGGGSGGGGSGGGGSGGGGSGGGGSGGGGSGGGGSEVQLVESGGGLVQPGGSLRLSCTFSGGTFSSYTMGWFRQAPGKEREFVAEVRWGGVTTYSNSLKDRFSISEDSVKNAVYLQMNSLKPEDTAVYYCAAVRQMYMTVVPDYWGQGTLVTVSS

SEQ ID NO: 438 - protein, 272 aa, Artificial Sequence
  Nanobody sequence
EVQLVESGGGLVQPGGSLRLSCAASGSVHKINFLGWYRQAPGKERELVATITIGDTTDYADSAKGRFTISRDEAKNMVYLQMNSLKPEDTAVYFCRAGSRLYPYNYWGQGTLVTVSSGGGGSGGGGSGGGGSGGGGSGGGGSGGGGSGGGGSEVQLVESGGGLVQPGGSLRLSCTFSGGTFSSYTMGWFRQAPGKEREFVAEVRWGGVTTYSNSLKDRFSISEDSVKNAVYLQMNSLKPEDTAVYYCAAVRQMYMTVVPDYWGQGTLVTVSS

SEQ ID NO: 439 - protein, 272 aa, Artificial Sequence; identical to SEQ ID NO: 425
  Nanobody sequence

SEQ ID NO: 440 - protein, 272 aa, Artificial Sequence
  Nanobody sequence
EVQLVESGGGLVQPGGSLRLSCAASGDVHKINILGWYRQAPAKEREMVAHITIGDATDYADSAKGRFTISRDEAKNMVYLQMNSLKPEDTAVYLCRAYSRIYPYNYWGQGTLVTVSSGGGGSGGGGSGGGGSGGGGSGGGGSGGGGSGGGGSEVQLVESGGGLVQPGGSLRLSCTFSGGTFSSYTMGWFRQAPGKEREFVAEVRWGGVTTYSNSLKDRFSISEDSVKNAVYLQMNSLKPEDTAVYYCAAVRQMYMTVVPDYWGQGTLVTVSS

SEQ ID NO: 441 - protein, 272 aa, Artificial Sequence
  Nanobody sequence
EVQLVESGGGLVQPGGSLRLSCTFSGGTFSSYTMGWFRQAPGKEREFVAEVRWGGVTTYSNSLKDRFSISEDSVKNAVYLQMNSLKPEDTAVYYCAAVRQMYMTVVPDYWGQGTLVTVSSGGGGSGGGGSGGGGSGGGGSGGGGSGGGGSGGGGSEVQLVESGGGLVQPGGSLRLSCVASGDVHKINFLGWYRQAPGKEREKVAHISIGDQTDYADSAKGRFTISRDESKNMVYLQMNSLKPEDTAVYFCRAFSRIYPYDYWGQGTLVTVSS

SEQ ID NO: 442 - protein, 272 aa, Artificial Sequence
  Nanobody sequence
EVQLVESGGGLVQPGGSLRLSCTFSGGTFSSYTMGWFRQAPGKEREFVAEVRWGGVTTYSNSLKDRFSISEDSVKNAVYLQMNSLKPEDTAVYYCAAVRQMYMTVVPDYWGQGTLVTVSSGGGGSGGGGSGGGGSGGGGSGGGGSGGGGSGGGGSEVQLVESGGGLVQPGGSLRLSCAASGEIGRINFYRWYRQAPGNQREVVATITIADKTDYADSAKGRFTISRDESRNMVYLQMSSLKPEDTAVYFCHAGSRLYPYDYWGQGTLVTVSS

SEQ ID NO: 443 - protein, 272 aa, Artificial Sequence
  Nanobody sequence
EVQLVESGGGLVQPGGSLRLSCTFSGGTFSSYTMGWFRQAPGKEREFVAEVRWGGVTTYSNSLKDRFSISEDSVKNAVYLQMNSLKPEDTAVYYCAAVRQMYMTVVPDYWGQGTLVTVSSGGGGSGGGGSGGGGSGGGGSGGGGSGGGGSGGGGSEVQLVESGGGLVQPGGSLRLSCVASGDVHKINFLGWYRQAPGKEREKVAHITIGDQADYADSAKGRFTISRDEAKNMVYLQMNSLKPEDTAVYFCRAGSRIYPYDYWGQGTLVTVSS

SEQ ID NO: 444 - protein, 272 aa, Artificial Sequence
  Nanobody sequence
EVQLVESGGGLVQPGGSLRLSCTFSGGTFSSYTMGWFRQAPGKEREFVAEVRWGGVTTYSNSLKDRFSISEDSVKNAVYLQMNSLKPEDTAVYYCAAVRQMYMTVVPDYWGQGTLVTVSSGGGGSGGGGSGGGGSGGGGSGGGGSGGGGSGGGGSEVQLVESGGGLVQPGGSLRLSCAASGDVHKINILGWYRQAPAKEREMVAHITIGDATDYADSAKGRFTISRDEAKNMVYLQMNSLKPEDTAVYFCRAYSRIYPYNYWGQGTLVTVSS

SEQ ID NO: 445 - protein, 272 aa, Artificial Sequence
  Nanobody sequence
EVQLVESGGGLVQPGGSLRLSCTFSGGTFSSYTMGWFRQAPGKEREFVAEVRWGGVTTYSNSLKDRFSISEDSVKNAVYLQMNSLKPEDTAVYYCAAVRQMYMTVVPDYWGQGTLVTVSSGGGGSGGGGSGGGGSGGGGSGGGGSGGGGSGGGGSEVQLVESGGGLVQPGGSLRLSCAASGSVHKINFLGWYRQAPGKERELVATITIGDTTDYADSAKGRFTISRDEAKNMVYLQMNSLKPEDTAVYFCRAGSRLYPYNYWGQGTLVTVSS

SEQ ID NO: 446 - protein, 272 aa, Artificial Sequence; identical to SEQ ID NO: 422
  Nanobody sequence

SEQ ID NO: 447 - protein, 272 aa, Artificial Sequence
  Nanobody sequence
EVQLVESGGGLVQPGGSLRLSCTFSGGTFSSYTMGWFRQAPGKEREFVAEVRWGGVTTYSNSLKDRFSISEDSVKNAVYLQMNSLKPEDTAVYYCAAVRQMYMTVVPDYWGQGTLVTVSSGGGGSGGGGSGGGGSGGGGSGGGGSGGGGSGGGGSEVQLVESGGGLVQPGGSLRLSCAASGDVYKINFLGWHRQAPGKEREKVAHITIGDATDYADSAKGRFTISRDEAKNMVYLQMNSLKPEDTAVYFCRAGSRIYPYDYWGQGTLVTVSS

SEQ ID NO: 448 - protein, 272 aa, Artificial Sequence
  Nanobody sequence
EVQLVESGGGLVQPGGSLRLSCTFSGGTFSSYTMGWFRQAPGKEREFVAEVRWGGVTTYSNSLKDRFSISEDSVKNAVYLQMNSLKPEDTAVYYCAAVRQMYMTVVPDYWGQGTLVTVSSGGGGSGGGGSGGGGSGGGGSGGGGSGGGGSGGGGSEVQLVESGGGLVQPGGSLRLSCAASGEVYKINFLGWYRQAPGKEREKVAHITIADAADYADFAKGRFTISRDEAKNMVYLQMNSLRPEDTAVYFCRAGSRIWPYDYWGQGTLVTVSS

SEQ ID NO: 449 - protein, 272 aa, Artificial Sequence
  Nanobody sequence
EVQLVESGGGLVQPGGSLRLSCTFSGGTFSSYTMGWFRQAPGKEREFVAEVRWGGVTTYSNSLKDRFSISEDSVKNAVYLQMNSLKPEDTAVYYCAAVRQMYMTVVPDYWGQGTLVTVSSGGGGSGGGGSGGGGSGGGGSGGGGSGGGGSGGGGSEVQLVESGGDLVQPGGSLRLSCAASGDVHKINFLGWYRQAPGKEREMVAHITIADATDYAEFAKGRFTISRDEPKNMVYLQMNSLKPEDTAVYLCRAGSRIYPYNYWGQGTLVTVSS

SEQ ID NO: 450 - protein, 272 aa, Artificial Sequence
  Nanobody sequence
EVQLVESGGGLVQPGGSLRLSCTFSGGTFSSYTMGWFRQAPGKEREFVAEVRWGGVTTYSNSLKDRFSISEDSVKNAVYLQMNSLKPEDTAVYYCAAVRQMYMTVVPDYWGQGTLVTVSSGGGGSGGGGSGGGGSGGGGSGGGGSGGGGSGGGGSEVQLVESGGGLVQPGGSLRLSCITSGETFKINIWGWYRQAPGKQRELVASLTIGGATNYADSVKGRFTISEDSAKNTVYLQMNSLKPEDTAVYFCNAKSRLYPYDYWGQGTLVTVSS

SEQ ID NO: 451 - protein, 272 aa, Artificial Sequence
  Nanobody sequence
EVQLVESGGGLVQPGGSLRLSCTFSGGTFSSYTMGWFRQAPGKEREFVAEVRWGGVTTYSNSLKDRFSISEDSVKNAVYLQMNSLKPEDTAVYYCAAVRQMYMTVVPDYWGQGTLVTVSSGGGGSGGGGSGGGGSGGGGSGGGGSGGGGSGGGGSEVQLVESGGGLVQPGGSLRLSCAASGSVHLLNFLGWYRQAPGKEREMVAHITIADATDYAHFAKGRFTISRDEAKNMVYLQMNSLRPEDTAVYFCRAGSRIYPYDYWGQGTLVTVSS

SEQ ID NO: 452 - protein, 272 aa, Artificial Sequence
  Nanobody sequence
EVQLVESGGGLVQPGGSLRLSCTFSGGTFSSYTMGWFRQAPGKEREFVAEVRWGGVTTYSNSLKDRFSISEDSVKNAVYLQMNSLKPEDTAVYYCAAVRQMYMTVVPDYWGQGTLVTVSSGGGGSGGGGSGGGGSGGGGSGGGGSGGGGSGGGGSEVQLVESGGGLVQPGGSLRLSCITSGETFKINIWGWYRQAPGKQRELVASLTIGGATDYADSVKGRFTISEDSAKNTVYLQMNSLKAEDTAVYFCNAKSRLYPYDYWGQGTLVTVSS

SEQ ID NO: 453 - protein, 272 aa, Artificial Sequence
  Nanobody sequence
EVQLVESGGGLVQPGGSLRLSCAASGDVHKINILGWYRQAPAKEREMVAHITIGDATSYADSAKGRFTISRDEAKNMVYLQLNNLKPEDTAVYFCRAYSRIYPYNYWGQGTLVTVSSGGGGSGGGGSGGGGSGGGGSGGGGSGGGGSGGGGSEVQLVESGGGLVQPGGSLRLSCTFSGGTFSSYTMGWFRQAPGKEREFVAEVRWGGVTTYSNSLKDRFSISEDSVKNAVYLQMNSLKPEDTAVYYCAAVRQMYMTVVPDYWGQGTLVTVSS

SEQ ID NO: 454 - protein, 272 aa, Artificial Sequence; identical to SEQ ID NO: 434
  Nanobody sequence

SEQ ID NO: 455 - protein, 272 aa, Artificial Sequence
  Nanobody sequence
EVQLVESGGGLVQPGGSLRLSCTFSGGTFSSYTMGWFRQAPGKEREFVAEVRWGGVTTYSNSLKDRFSISEDSVKNAVYLQMNSLKPEDTAVYYCAAVRQMYMTVVPDYWGQGTLVTVSSGGGGSGGGGSGGGGSGGGGSGGGGSGGGGSGGGGSEVQLVESGGGLVQPGGSLRLSCAASGDVHKINILGWYRQAPAKEREMVAHITIGDATSYADSAKGRFTISRDEAKNMVYLQLNNLKPEDTAVYFCRAYSRIYPYNYWGQGTLVTVSS

SEQ ID NO: 456 - protein, 272 aa, Artificial Sequence; identical to SEQ ID NO: 441
  Nanobody sequence

SEQ ID NO: 457 - protein, 272 aa, Artificial Sequence
  Nanobody sequence
EVQLVESGGDLVQPGGSLRLSCAASGDVHKINFLGWYRQAPGKEREMVAHITIADATDYAEFAKGRFTISRDEPKNMVYLQMNSLKPEDTAVYLCRAGSRIYPYNYWGQGTLVTVSSGGGGSGGGGSGGGGSGGGGSGGGGSGGGGSGGGGSEVQLVESGGGLVQPGGSLRLSCTFSGGTFSSYTMGWFRQAPGKEREFVAEVRWGGVTTYSNSLKDRFSISEDSVKNAVYLQMNSLKPEDTAVYYCAAVRQMYMTVVPDYWGQGTLVTVSS

SEQ ID NO: 458 - protein, 272 aa, Artificial Sequence
  Nanobody sequence
EVQLVESGGGLVQPGGSLRLSCTFSGGTFSSYTMGWFRQAPGKEREFVAEVRWGGVTTYSNSLKDRFSISEDSVKNAVYLQMNSLKPEDTAVYYCAAVRQMYMTVVPDYWGQGTLVTVSSGGGGSGGGGSGGGGSGGGGSGGGGSGGGGSGGGGSEVQLVESGGGLVQPGGSLRLSCAASGDVHKINILGWYRQAPAKEREMVAHITIGDATDYADSAKGRFTISRDEAKNMVYLQMNSLKPEDTAVYLCRAYSRIYPYNYWGQGTLVTVSS

SEQ ID NO: 459 - protein, 272 aa, Artificial Sequence
  Nanobody sequence
EVQLVESGGGLVQPGGSLRLSCTFSGGTFSSYTMGWFRQAPGKEREFVAEVRWGGVTTYSNSLKDRFSISEDSVKNAVYLQMNSLKPEDTAVYYCAAVRQMYMTVVPDYWGQGTLVTVSSGGGGSGGGGSGGGGSGGGGSGGGGSGGGGSGGGGSEVQLVESGGGLVQPGGSLKLSCAASGAVHKINFLGWYRQTPEKEREMVATITIGDEVDYADSAKGRFTISRDEAKNMVYLQMTSLKPEDTAVYVCRAGSRLYPYNYWGQGTLVTVSS

SEQ ID NO: 460 - protein, 422 aa, Artificial Sequence
  Nanobody sequence
EVQLVESGGGLVQPGGSLRLSCTFSGGTFSSYTMGWFRQAPGKEREFVAEVRWGGVTTYSNSLKDRFSISEDSVKNAVYLQMNSLKPEDTAVYYCAAVRQMYMTVVPDYWGQGTLVTVSSGGGGSGGGGSGGGGSGGGGSGGGGSGGGGSGGGGSEVQLVESGGGLVQPGGSLRLSCVASGDVHKINFLGWYRQAPGKEREKVAHISIGDQTDYADSAKGRFTISRDESKNMVYLQMNSLKPEDTAVYFCRAFSRIYPYDYWGQGTLVTVSSGGGGSGGGGSGGGGSGGGGSGGGGSGGGGSGGGGSEVQLVESGGGLVQPGNSLRLSCAASGFTFSSFGMSWVRQAPGKGLEWVSSISGSGSDTLYADSVKGRFTISRDNAKTTLYLQMNSLRPEDTAVYYCTIGGSLSRSSQGTLVTVSS

SEQ ID NO: 461 - protein, 422 aa, Artificial Sequence
  Nanobody sequence
EVQLVESGGGLVQPGGSLRLSCTFSGGTFSSYTMGWFRQAPGKEREFVAEVRWGGVTTYSNSLKDRFSISEDSVKNAVYLQMNSLKPEDTAVYYCAAVRQMYMTVVPDYWGQGTLVTVSSGGGGSGGGGSGGGGSGGGGSGGGGSGGGGSGGGGSEVQLVESGGGLVQPGGSLRLSCITSGETFKINIWGWYRQAPGKQRELVASLTIGGATNYADSVKGRFTISEDSAKNTVYLQMNSLKPEDTAVYFCNAKSRLYPYDYWGQGTLVTVSSGGGGSGGGGSGGGGSGGGGSGGGGSGGGGSGGGGSEVQLVESGGGLVQPGNSLRLSCAASGFTFSSFGMSWVRQAPGKGLEWVSSISGSGSDTLYADSVKGRFTISRDNAKTTLYLQMNSLRPEDTAVYYCTIGGSLSRSSQGTLVTVSS

SEQ ID NO: 462 - protein, 270 aa, Artificial Sequence
  Nanobody sequence
EVQLVESGGGLVQAGGSLRLSCAASGITFSINTMGWYRQAPGKQRELVALISSIGDTYYADSVKGRFTISRDNAKNTVYLQMNSLKPEDTAVYYCKRFRTAAQGTDYWGQGTLVTVSSGGGGSGGGGSGGGGSGGGGSGGGGSGGGGSGGGGSEVQLVESGGGLVQPGGSLRLSCVASGDVHKINFLGWYRQAPGKEREKVAHISIGDQTDYADSAKGRFTISRDESKNMVYLQMNSLKPEDTAVYFCRAFSRIYPYDYWGQGTLVTVSS

SEQ ID NO: 463 - protein, 270 aa, Artificial Sequence
  Nanobody sequence
EVQLVESGGGLVQPGGSLRLSCVASGDVHKINFLGWYRQAPGKEREKVAHISIGDQTDYADSAKGRFTISRDESKNMVYLQMNSLKPEDTAVYFCRAFSRIYPYDYWGQGTLVTVSSGGGGSGGGGSGGGGSGGGGSGGGGSGGGGSGGGGSEVQLVESGGGLVQAGGSLRLSCAASGITFSINTMGWYRQAPGKQRELVALISSIGDTYYADSVKGRFTISRDNAKNTVYLQMNSLKPEDTAVYYCKRFRTAAQGTDYWGQGTLVTVSS

SEQ ID NO: 464 - protein, 439 aa, Artificial Sequence
  Nanobody sequence
EVQLVESGGGLVQAGGSLRLSCAASGRTFSSYVMGWFRQATGKEREFVATIAWDSGSTYYADSVKGRFTISRDNAKNTVHLQMNSLKPEDTAVYYCAASYNVYYNNYYYPISRDEYDYWGQGTLVTVSSGGGGSGGGGSGGGGSGGGGSGGGGSGGGGSGGGGSEVQLVESGGGSVQAGGSLRLSCAASGDTYGSYWMGWFRQAPGKEREGVAAINRGGGYTVYADSVKGRFTISRDTAKNTVYLQMNSLRPDDTADYYCAASGVLGGLHEDWFNYWGQGTLVTVSSGGGGSGGGGSGGGGSGGGGSGGGGSGGGGSGGGGSEVQLVESGGGLVQPGGSLRLSCVASGDVHKINFLGWYRQAPGKEREKVAHISIGDQTDYADSAKGRFTISRDESKNMVYLQMNSLKPEDTAVYFCRAFSRIYPYDYWGQGTLVTVSS

SEQ ID NO: 465 - protein, 443 aa, Artificial Sequence
  Nanobody sequence
EVQLVESGGGSVQAGGSLRLSCAASGYTIGPYCMGWFRQAPGKEREGVAAINMGGGITYYADSVKGRFTISQDNAKNTVYLLMNSLEPEDTAIYYCAADSTIYASYYECGHGLSTGGYGYDSWGQGTLVTVSSGGGGSGGGGSGGGGSGGGGSGGGGSGGGGSGGGGSEVQLVESGGGSVQAGGSLRLSCAASGDTYGSYWMGWFRQAPGKEREGVAAINRGGGYTVYADSVKGRFTISRDTAKNTVYLQMNSLRPDDTADYYCAASGVLGGLHEDWFNYWGQGTLVTVSSGGGGSGGGGSGGGGSGGGGSGGGGSGGGGSGGGGSEVQLVESGGGLVQPGGSLRLSCVASGDVHKINFLGWYRQAPGKEREKVAHISIGDQTDYADSAKGRFTISRDESKNMVYLQMNSLKPEDTAVYFCRAFSRIYPYDYWGQGTLVTVSS

SEQ ID NO: 466 - protein, 449 aa, Artificial Sequence
  Nanobody sequence
EVQLVESGGGLVQAGGSLRLSCAASGRTFSSYVMGWFRQATGKEREFVATIAWDSGSTYYADSVKGRFTISRDNAKNTVHLQMNSLKPEDTAVYYCAASYNVYYNNYYYPISRDEYDYWGQGTLVTVSSGGGGSGGGGSGGGGSGGGGSGGGGSGGGGSGGGGSEVQLVESGGGSVQAGGSLRLSCAASGYTIGPYCMGWFRQAPGKEREGVAAINMGGGITYYADSVKGRFTISQDNAKNTVYLLMNSLEPEDTAIYYCAADSTIYASYYECGHGLSTGGYGYDSWGQGTLVTVSSGGGGSGGGGSGGGGSGGGGSGGGGSGGGGSGGGGSEVQLVESGGGLVQPGGSLRLSCVASGDVHKINFLGWYRQAPGKEREKVAHISIGDQTDYADSAKGRFTISRDESKNMVYLQMNSLKPEDTAVYFCRAFSRIYPYDYWGQGTLVTVSS

SEQ ID NO: 467 - protein, 422 aa, Artificial Sequence
  Nanobody sequence
DVQLVESGGGLVQPGGSLRLSCTFSGGTFSSYTMGWFRQAPGKEREFVAEVRWGGVTTYSNSLKDRFSISEDSVKNAVYLQMNSLKPEDTAVYYCAAVRQMYMTVVPDYWGQGTLVTVSSGGGGSGGGGSGGGGSGGGGSGGGGSGGGGSGGGGSEVQLVESGGGLVQPGGSLRLSCAASGDVHKINILGWYRQAPAKEREMVAHITIGDATDYADSAKGRFTISRDEAKNMVYLQMNSLKPEDTAVYFCRAYSRIYPYNYWGQGTLVTVSSGGGGSGGGGSGGGGSGGGGSGGGGSGGGGSGGGGSEVQLVESGGGLVQPGNSLRLSCAASGFTFSSFGMSWVRQAPGKGLEWVSSISGSGSDTLYADSVKGRFTISRDNAKTTLYLQMNSLRPEDTAVYYCTIGGSLSRSSQGTLVTVSS

SEQ ID NO: 468 - protein, 272 aa, Artificial Sequence
  Nanobody sequence
DVQLVESGGGLVQPGGSLRLSCTFSGGTFSSYTMGWFRQAPGKEREFVAEVRWGGVTTYSNSLKDRFSISEDSVKNAVYLQMNSLKPEDTAVYYCAAVRQMYMTVVPDYWGQGTLVTVSSGGGGSGGGGSGGGGSGGGGSGGGGSGGGGSGGGGSEVQLVESGGGLVQPGGSLRLSCVASGDVHKINFLGWYRQAPGKEREKVAHISIGDQTDYADSAKGRFTISRDESKNMVYLQMNSLKPEDTAVYFCRAFSRIYPYDYWGQGTLVTVSS

SEQ ID NO: 469 - protein, 429 aa, Artificial Sequence
  Nanobody sequence
DVQLVESGGGLVQAGDSLRLSCAASGRTFSSYAMGWFRQAPGKEREFVAAISWSDGSTYYADSVKGRFTISRDNAKNTVYLQMNSLKPEDTAVYYCAADLTSTNPGSYIYIWAYDYWGQGTQVTVSSGGGGSGGGGSGGGGSGGGGSGGGGSGGGGSGGGGSEVQLVESGGGLVQPGGSLRLSCAASGDVHKINILGWYRQAPAKEREMVAHITIGDATDYADSAKGRFTISRDEAKNMVYLQMNSLKPEDTAVYFCRAYSRIYPYNYWGQGTLVTVSSGGGGSGGGGSGGGGSGGGGSGGGGSGGGGSGGGGSEVQLVESGGGLVQPGNSLRLSCAASGFTFSSFGMSWVRQAPGKGLEWVSSISGSGSDTLYADSVKGRFTISRDNAKTTLYLQMNSLRPEDTAVYYCTIGGSLSRSSQGTLVTVSS

SEQ ID NO: 470 - protein, 272 aa, Artificial Sequence
  Nanobody sequence
DVQLVESGGGLVQPGGSLRLSCTFSGGTFSSYTMGWFRQAPGKEREFVAEVRWGGVTTYSNSLKDRFSISEDSVKNAVYLQMNSLKPEDTAVYYCAAVRQMYMTVVPDYWGQGTLVTVSSGGGGSGGGGSGGGGSGGGGSGGGGSGGGGSGGGGSEVQLVESGGGLVQPGGSLRLSCAASGDVHKINILGWYRQAPAKEREMVAHITIGDATDYADSAKGRFTISRDEAKNMVYLQMNSLKPEDTAVYFCRAYSRIYPYNYWGQGTLVTVSS

SEQ ID NO: 471 - protein, 279 aa, Artificial Sequence
  Nanobody sequence
DVQLVESGGGLVQAGDSLRLSCAASGRTFSSYAMGWFRQAPGKEREFVAAISWSDGSTYYADSVKGRFTISRDNAKNTVYLQMNSLKPEDTAVYYCAADLTSTNPGSYIYIWAYDYWGQGTQVTVSSGGGGSGGGGSGGGGSGGGGSGGGGSGGGGSGGGGSEVQLVESGGGLVQPGGSLRLSCAASGDVHKINILGWYRQAPAKEREMVAHITIGDATDYADSAKGRFTISRDEAKNMVYLQMNSLKPEDTAVYFCRAYSRIYPYNYWGQGTLVTVSS

SEQ ID NO: 472 - protein, 10 aa, Artificial Sequence
  CDR1
GFTFSSFGMS

SEQ ID NO: 473 - protein, 10 aa, Artificial Sequence
  CDR1
GFTFRSFGMS

SEQ ID NO: 474 - protein, 10 aa, Artificial Sequence
  CDR2
SISGSGSDTL

SEQ ID NO: 475 - protein, 6 aa, Artificial Sequence
  CDR3
GGSLSR

SEQ ID NO: 476 - protein, 110 aa, Homo sapiens
NAGVTQTPKFRILKIGQSMTLQCTQDMNHNYMYWYRQDPGMGLKLIYYSVGAGITDKGEVPNGYNVSRSTTEDFPLRLELAAPSQTSVYFCASTYHGTGYFGEGSWLTVV

SEQ ID NO: 477 - protein, 112 aa, Homo sapiens
DGGITQSPKYLFRKEGQNVTLSCEQNLNHDAMYWYRQDPGQGLRLIYYSQIVNDFQKGDIAEGYSVSREKKESFPLTVTSAQKNPTAFYLCASSSRSSYEQYFGPGTRLTVT

SEQ ID NO: 478 - protein, 114 aa, Homo sapiens
VVSQHPSWVIAKSGTSVKIECRSLDFQATTMFWYRQFPKQSLMLMATSNEGSKATYEQGVEKDKFLINHASLTLSTLTVTSAHPEDSSFYICSARGGSYNSPLHFGNGTRLTVT

SEQ ID NO: 479 - protein, 96 aa, Homo sapiens
PNIQNPDPAVYQLRDSKSSDKSVCLFTDFDSQTNVSQSKDSDVYITDKTVLDMRSMDFKSNSAVAWSNKSDFACANAFNNSIIPEDTFFPSPESSC

SEQ ID NO: 480 - protein, 131 aa, Homo sapiens
EDLNKVFPPEVAVFEPSEAEISHTQKATLVCLATGFFPDHVELSWWVNGKEVHSGVSTDPQPLKEQPALNDSRYCLSSRLRVSATFWQNPRNHFRCQVQFYGLSENDEWTQDRAKPVTQIVSAEAWGRADC

SEQ ID NO: 481 - protein, 5 aa, Artificial Sequence
  CDR1
SFGMS

SEQ ID NO: 482 - protein, 17 aa, Artificial Sequence
  CDR2
SISGSGSDTLYADSVKG

SEQ ID NO: 483 - protein, 98 aa, Artificial Sequence
  Nanobody sequence
QVQLVESGGGLVQPGGSLRLSCAASGFTLDYYAIGWFRQAPGKEREGVSCISSSDGSTYYADSVKGRFTISRDNAKNTVYLQMNSLKPEDTAVYYCAA

SEQ ID NO: 484 - protein, 142 aa, Homo sapiens
PNIQNPDPAVYQLRDSKSSDKSVCLFTDFDSQTNVSQSKDSDVYITDKTVLDMRSMDFKSNSAVAWSNKSDFACANAFNNSIIPEDTFFPSPESSCDVKLVEKSFETDTNLNFQNLSVIGFRILLLKVAGFNLLMTLRLWSS

SEQ ID NO: 485 - protein, 177 aa, Homo sapiens
EDLNKVFPPEVAVFEPSEAEISHTQKATLVCLATGFFPDHVELSWWVNGKEVHSGVSTDPQPLKEQPALNDSRYCLSSRLRVSATFWQNPRNHFRCQVQFYGLSENDEWTQDRAKPVTQIVSAEAWGRADCGFTSVSYQQGVLSATILYEILLGKATLYAVLVSALVLMAMVKRKDF

SEQ ID NO: 486 - protein, 623 aa, Artificial Sequence
  Nanobody sequence
EVQLVESGGGLVQAGGSLRLSCAASGRTFSSYVMGWFRQATGKEREFVATIAWDSGSTYYADSVKGRFTISRDNAKNTVHLQMNSLKPEDTAVYYCAASYNVYYNNYYYPISRDEYDYWGQGTLVTVSSGGGGSGGGGSGGGGSGGGGSGGGGSGGGGSGGGGSEVQLVESGGGSVQAGGSLRLSCAASGDTYGSYWMGWFRQAPGKEREGVAAINRGGGYTVYADSVKGRFTISRDTAKNTVYLQMNSLRPDDTADYYCAASGVLGGLHEDWFNYWGQGTLVTVSSGGGGSGGGGSGGGGSGGGGSGGGGSGGGGSGGGGSEVQLVESGGGLVQPGGSLRLSCVASGDVHKINFLGWYRQAPGKEREKVAHISIGDQTDYADSAKGRFTISRDESKNMVYLQMNSLKPEDTAVYFCRAFSRIYPYDYWGQGTLVTVSSGGGGSGGGGSGGGGSGGGGSGGGGSGGGGSGGGGSEVQLVESGGGLVQPGNSLRLSCAASGFTFSSFGMSWVRQAPGKGLEWVSSISGSGSDTLYADSVKGRFTISRDNAKTTLYLQMNSLRPEDTAVYYCTIGGSLSRSSQGTLVTVSSGAADYKDHDGDYKDHDIDYKDDDDKGAAHHHHHH

SEQ ID NO: 487 - protein, 589 aa, Artificial Sequence
  Nanobody sequence
EVQLVESGGGLVQAGGSLRLSCAASGRTFSSYVMGWFRQATGKEREFVATIAWDSGSTYYADSVKGRFTISRDNAKNTVHLQMNSLKPEDTAVYYCAASYNVYYNNYYYPISRDEYDYWGQGTLVTVSSGGGGSGGGGSGGGGSGGGGSGGGGSGGGGSGGGGSEVQLVESGGGSVQAGGSLRLSCAASGDTYGSYWMGWFRQAPGKEREGVAAINRGGGYTVYADSVKGRFTISRDTAKNTVYLQMNSLRPDDTADYYCAASGVLGGLHEDWFNYWGQGTLVTVSSGGGGSGGGGSGGGGSGGGGSGGGGSGGGGSGGGGSEVQLVESGGGLVQPGGSLRLSCVASGDVHKINFLGWYRQAPGKEREKVAHISIGDQTDYADSAKGRFTISRDESKNMVYLQMNSLKPEDTAVYFCRAFSRIYPYDYWGQGTLVTVSSGGGGSGGGGSGGGGSGGGGSGGGGSGGGGSGGGGSEVQLVESGGGLVQPGNSLRLSCAASGFTFSSFGMSWVRQAPGKGLEWVSSISGSGSDTLYADSVKGRFTISRDNAKTTLYLQMNSLRPEDTAVYYCTIGGSLSRSSQGTLVTVSS